European Patent Application EP 4 257 193 A2, published October 11, 2023. Title: TRISPECIFIC AND/OR TRIVALENT BINDING PROTEINS. Applicant: Sanofi. Application EP. The sequence listing filed with the application follows.

SEQUENCE LISTING (179 sequences)

SEQ ID NO: 1 - protein, 447 aa, synthetic construct
  REGION 1..447: note = Synthetic Construct
EVQLVESGGGLVQPGGSLRLSCAASGFNIKDTYIHWVRQAPGKGLEWVARIYPTNGYTRYADSVKGRFTISADTSKNTAYLQMNSLRAEDTAVYYCSRWGGDGFYAMDYWGQGTLVTVSSASTKGPSVFPLAPCSRSTSESTAALGCLVKDYFPEPVTVSWNSGALTSGVHTFPAVLQSSGLYSLSSVVTVPSSSLGTKTYTCNVDHKPSNTKVDKRVESKYGPPCPPCPAPEFLGGPSVFLFPPKPKDTLMISRTPEVTCVVVDVSQEDPEVQFNWYVDGVEVHNAKTKPREEQFNSTYRVVSVLTVLHQDWLNGKEYKCKVSNKGLPSSIEKTISKAKGQPREPQVYTLPPCQEEMTKNQVSLWCLVKGFYPSDIAVEWESNGQPENNYKTTPPVLDSDGSFFLYSKLTVDKSRWQEGNVFSCSVMHEALHNHYTQKSLSLSLGK

SEQ ID NO: 2 - protein, 214 aa, synthetic construct
  REGION 1..214: note = Synthetic Construct
DIQMTQSPSSLSASVGDRVTITCRASQDVNTAVAWYQQKPGKAPKLLIYSASFLYSGVPSRFSGSRSGTDFTLTISSLQPEDFATYYCQQHYTTPPTFGQGTKVEIKRTVAAPSVFIFPPSDEQLKSGTASVVCLLNNFYPREAKVQWKVDNALQSGNSQESVTEQDSKDSTYSLSSTLTLSKADYEKHKVYACEVTHQGLSSPVTKSFNRGEC

SEQ ID NO: 3 - protein, 571 aa, synthetic construct
  REGION 1..571: note = Synthetic Construct
QVQLVQSGAEVVKPGASVKVSCKASGYTFTSYYIHWVRQAPGQGLEWIGSIYPGNVNTNYAQKFQGRATLTVDTSISTAYMELSRLRSDDTAVYYCTRSHYGLDWNFDVWGKGTTVTVSSSQVQLVESGGGVVQPGRSLRLSCAASGFTFTKAWMHWVRQAPGKQLEWVAQIKDKSNSYATYYADSVKGRFTISRDDSKNTLYLQMNSLRAEDTAVYYCRGVYYALSPFDYWGQGTLVTVSSRTASTKGPSVFPLAPCSRSTSESTAALGCLVKDYFPEPVTVSWNSGALTSGVHTFPAVLQSSGLYSLSSVVTVPSSSLGTKTYTCNVDHKPSNTKVDKRVESKYGPPCPPCPAPEFLGGPSVFLFPPKPKDTLMISRTPEVTCVVVDVSQEDPEVQFNWYVDGVEVHNAKTKPREEQFNSTYRVVSVLTVLHQDWLNGKEYKCKVSNKGLPSSIEKTISKAKGQPREPQVCTLPPSQEEMTKNQVSLSCAVKGFYPSDIAVEWESNGQPENNYKTTPPVLDSDGSFFLVSKLTVDKSRWQEGNVFSCSVMHEALHNHYTQKSLSLSLGK

SEQ ID NO: 4 - protein, 338 aa, synthetic construct
  REGION 1..338: note = Synthetic Construct
DIVMTQTPLSLSVTPGQPASISCKSSQSLVHNNANTYLSWYLQKPGQSPQSLIYKVSNRFSGVPDRFSGSGSGTDFTLKISRVEAEDVGVYYCGQGTQYPFTFGSGTKVEIKGQPKAAPDIQMTQSPSSLSASVGDRVTITCQASQNIYVWLNWYQQKPGKAPKLLIYKASNLHTGVPSRFSGSGSGTDFTLTISSLQPEDIATYYCQQGQTYPYTFGQGTKLEIKTKGPSRTVAAPSVFIFPPSDEQLKSGTASVVCLLNNFYPREAKVQWKVDNALQSGNSQESVTEQDSKDSTYSLSSTLTLSKADYEKHKVYACEVTHQGLSSPVTKSFNRGEC

SEQ ID NO: 5 - DNA, 1341 bp, synthetic construct
  misc_feature 1..1341: note = Synthetic Construct
  source 1..1341: mol_type = other DNA
gaagtgcagctggtggaatctggcggcggactggtgcagcctggcggatctctgagactgagctgtgccgccagcggcttcaacatcaaggacacctacatccactgggtgcgccaggcccctggcaagggactggaatgggtggccagaatctaccccaccaacggctacaccagatacgccgacagcgtgaagggccggttcaccatcagcgccgacaccagcaagaacaccgcctacctgcagatgaacagcctgcgggccgaggacaccgccgtgtactactgtagtagatggggaggcgacggcttctacgccatggactattggggccagggcaccctcgtgaccgtgtctagtgcgtcgaccaagggcccatcggtgttccctctggccccttgcagcagaagcaccagcgaatctacagccgccctgggctgcctcgtgaaggactactttcccgagcccgtgaccgtgtcctggaactctggcgctctgacaagcggcgtgcacacctttccagccgtgctccagagcagcggcctgtactctctgagcagcgtcgtgacagtgcccagcagcagcctgggcaccaagacctacacctgtaacgtggaccacaagcccagcaacaccaaggtggacaagcgggtggaatctaagtacggccctccctgccctccttgcccagcccctgaatttctgggcggaccctccgtgttcctgttccccccaaagcccaaggacaccctgatgatcagccggacccccgaagtgacctgcgtggtggtggatgtgtcccaggaagatcccgaggtgcagttcaattggtacgtggacggcgtggaagtgcacaacgccaagaccaagcccagagaggaacagttcaacagcacctaccgggtggtgtccgtgctgaccgtgctgcaccaggactggctgaacggcaaagagtacaagtgcaaggtgtccaacaagggcctgcccagctccatcgagaaaaccatcagcaaggccaagggccagccccgcgagcctcaagtgtataccctgcccccttgccaggaagagatgaccaagaaccaggtgtccctgtggtgtctcgtgaaaggcttctaccccagcgacattgccgtggaatgggagagcaacggccagcccgagaacaactacaagaccaccccccctgtgctggacagcgacggctcattcttcctgtactccaagctgaccgtggacaagagccggtggcaggaaggcaacgtgttcagctgctccgtgatgcacgaggccctgcacaaccactacacccagaagtccctgtctctgtccctgggcaag

SEQ ID NO: 6 - DNA, 642 bp, synthetic construct
  misc_feature 1..642: note = Synthetic Construct
  source 1..642: mol_type = other DNA
gacatccagatgacccagagccccagcagcctgtctgccagcgtgggcgacagagtgaccatcacctgtagagccagccaggacgtgaacaccgccgtggcctggtatcagcagaagcctggcaaggcccccaagctgctgatctacagcgccagcttcctgtacagcggcgtgcccagcagattcagcggaagcagaagcggcaccgacttcaccctgaccatcagctccctgcagcccgaggacttcgccacctactactgccagcagcactacaccaccccccccacatttggccagggcaccaaggtggaaatcaagcgtacggtggccgctcccagcgtgttcatcttcccacctagcgacgagcagctgaagtccggcacagcctctgtcgtgtgcctgctgaacaacttctacccccgcgaggccaaagtgcagtggaaggtggacaacgccctgcagagcggcaacagccaggaaagcgtgaccgagcaggacagcaaggactccacctacagcctgagcagcaccctgacactgagcaaggccgactacgagaagcacaaggtgtacgcctgcgaagtgacccaccagggcctgtctagccccgtgaccaagagcttcaaccggggcgagtgt

SEQ ID NO: 7 - DNA, 1713 bp, synthetic construct
  misc_feature 1..1713: note = Synthetic Construct
  source 1..1713: mol_type = other DNA
caggtgcagctggtgcagtctggcgccgaggtcgtgaaacctggcgcctctgtgaaggtgtcctgcaaggccagcggctacacctttaccagctactacatccactgggtgcgccaggcccctggacagggactggaatggatcggcagcatctaccccggcaacgtgaacaccaactacgcccagaagttccagggcagagccaccctgaccgtggacaccagcatcagcaccgcctacatggaactgagccggctgagaagcgacgacaccgccgtgtactactgcacccggtcccactacggcctggattggaacttcgacgtgtggggcaagggcaccaccgtgacagtgtctagcagccaggtgcagctggtggaatctggcggcggagtggtgcagcctggcagaagcctgagactgagctgtgccgccagcggcttcaccttcaccaaggcctggatgcactgggtgcgccaggcccctggaaagcagctggaatgggtggcccagatcaaggacaagagcaacagctacgccacctactacgccgacagcgtgaagggccggttcaccatcagccgggacgacagcaagaacaccctgtacctgcagatgaacagcctgcgggccgaggacaccgccgtgtactactgtcggggcgtgtactatgccctgagccccttcgattactggggccagggaaccctcgtgaccgtgtctagtcggaccgccagcacaaagggcccatcggtgttccctctggccccttgcagcagaagcaccagcgaatctacagccgccctgggctgcctcgtgaaggactactttcccgagcccgtgaccgtgtcctggaactctggcgctctgacaagcggcgtgcacacctttccagccgtgctccagagcagcggcctgtactctctgagcagcgtcgtgacagtgcccagcagcagcctgggcaccaagacctacacctgtaacgtggaccacaagcccagcaacaccaaggtggacaagcgggtggaatctaagtacggccctccctgccctccttgcccagcccctgaatttctgggcggaccctccgtgttcctgttccccccaaagcccaaggacaccctgatgatcagccggacccccgaagtgacctgcgtggtggtggatgtgtcccaggaagatcccgaggtgcagttcaattggtacgtggacggcgtggaagtgcacaacgccaagaccaagcccagagaggaacagttcaacagcacctaccgggtggtgtccgtgctgaccgtgctgcaccaggactggctgaacggcaaagagtacaagtgcaaggtgtccaacaagggcctgcccagctccatcgagaaaaccatcagcaaggccaagggccagccccgcgagcctcaagtgtgtaccctgccccctagccaggaagagatgaccaagaaccaggtgtccctgagctgtgccgtgaaaggcttctaccccagcgacattgccgtggaatgggagagcaacggccagcccgagaacaactacaagaccaccccccctgtgctggacagcgacggctcattcttcctggtgtccaagctgaccgtggacaagagccggtggcaggaaggcaacgtgttcagctgctccgtgatgcacgaggccctgcacaaccactacacccagaagtccctgtctctgtccctgggcaag

SEQ ID NO: 8 - DNA, 1014 bp, synthetic construct
  misc_feature 1..1014: note = Synthetic Construct
  source 1..1014: mol_type = other DNA
gacatcgtgatgacccagacccccctgagcctgagcgtgacacctggacagcctgccagcatcagctgcaagagcagccagagcctggtgcacaacaacgccaacacctacctgagctggtatctgcagaagcccggccagagcccccagtccctgatctacaaggtgtccaacagattcagcggcgtgcccgacagattctccggcagcggctctggcaccgacttcaccctgaagatcagccgggtggaagccgaggacgtgggcgtgtactattgtggccagggcacccagtaccccttcacctttggcagcggcaccaaggtggaaatcaagggccagcccaaggccgcccccgacatccagatgacccagagccccagcagcctgtctgccagcgtgggcgacagagtgaccatcacctgtcaggccagccagaacatctacgtgtggctgaactggtatcagcagaagcccggcaaggcccccaagctgctgatctacaaggccagcaacctgcacaccggcgtgcccagcagattttctggcagcggctccggcaccgacttcaccctgacaatcagctccctgcagcccgaggacattgccacctactactgccagcagggccagacctacccctacacctttggccagggcaccaagctggaaatcaagaccaagggccccagccgtacggtggccgctcccagcgtgttcatcttcccacctagcgacgagcagctgaagtccggcacagcctctgtcgtgtgcctgctgaacaacttctacccccgcgaggccaaagtgcagtggaaggtggacaacgccctgcagagcggcaacagccaggaaagcgtgaccgagcaggacagcaaggactccacctacagcctgagcagcaccctgacactgagcaaggccgactacgagaagcacaaggtgtacgcctgcgaagtgacccaccagggcctgtctagccccgtgaccaagagcttcaaccggggcgagtgt

SEQ ID NO: 9 - protein, 571 aa, synthetic construct
  REGION 1..571: note = Synthetic Construct
QVQLQESGPGLVKPSQTLSLTCTVSGFSLSDYGVHWVRQPPGKGLEWLGVIWAGGGTNYNPSLKSRKTISKDTSKNQVSLKLSSVTAADTAVYYCARDKGYSYYYSMDYWGQGTTVTVSSSQVQLVESGGGVVQPGRSLRLSCAASGFTFTKAWMHWVRQAPGKQLEWVAQIKDKSNSYATYYADSVKGRFTISRDDSKNTLYLQMNSLRAEDTAVYYCRGVYYALSPFDYWGQGTLVTVSSRTASTKGPSVFPLAPCSRSTSESTAALGCLVKDYFPEPVTVSWNSGALTSGVHTFPAVLQSSGLYSLSSVVTVPSSSLGTKTYTCNVDHKPSNTKVDKRVESKYGPPCPPCPAPEFLGGPSVFLFPPKPKDTLMISRTPEVTCVVVDVSQEDPEVQFNWYVDGVEVHNAKTKPREEQFNSTYRVVSVLTVLHQDWLNGKEYKCKVSNKGLPSSIEKTISKAKGQPREPQVCTLPPSQEEMTKNQVSLSCAVKGFYPSDIAVEWESNGQPENNYKTTPPVLDSDGSFFLVSKLTVDKSRWQEGNVFSCSVMHEALHNHYTQKSLSLSLGK

SEQ ID NO: 10 - protein, 342 aa, synthetic construct
  REGION 1..342: note = Synthetic Construct
DIVMTQTPLSLSVTPGQPASISCKSSQSLVHNNANTYLSWYLQKPGQSPQSLIYKVSNRFSGVPDRFSGSGSGTDFTLKISRVEAEDVGVYYCGQGTQYPFTFGSGTKVEIKGQPKAAPDIVLTQSPASLAVSPGQRATITCRASESVEYYVTSLMQWYQQKPGQPPKLLIFAASNVESGVPARFSGSGSGTDFTLTINPVEANDVANYYCQQSRKVPYTFGQGTKLEIKTKGPSRTVAAPSVFIFPPSDEQLKSGTASVVCLLNNFYPREAKVQWKVDNALQSGNSQESVTEQDSKDSTYSLSSTLTLSKADYEKHKVYACEVTHQGLSSPVTKSFNRGEC

SEQ ID NO: 11 - DNA, 1713 bp, synthetic construct
  misc_feature 1..1713: note = Synthetic Construct
  source 1..1713: mol_type = other DNA
caggtgcagctgcaggaatctggccctggcctcgtgaagcctagccagaccctgagcctgacctgtaccgtgtccggcttcagcctgagcgactacggcgtgcactgggtgcgccagccacctggaaaaggcctggaatggctgggcgtgatctgggctggcggaggcaccaactacaaccccagcctgaagtccagaaagaccatcagcaaggacaccagcaagaaccaggtgtccctgaagctgagcagcgtgacagccgccgataccgccgtgtactactgcgccagagacaagggctacagctactactacagcatggactactggggccagggcaccaccgtgaccgtgtcatcctctcaggtgcagctggtggaatctggcggcggagtggtgcagcctggcagaagcctgagactgagctgtgccgccagcggcttcaccttcaccaaggcctggatgcactgggtgcgccaggcccctggaaagcagctggaatgggtggcccagatcaaggacaagagcaacagctacgccacctactacgccgacagcgtgaagggccggttcaccatcagccgggacgacagcaagaacaccctgtacctgcagatgaacagcctgcgggccgaggacaccgccgtgtactactgtcggggcgtgtactatgccctgagccccttcgattactggggccagggaaccctcgtgaccgtgtctagtcggaccgcttcgaccaagggcccatcggtgttccctctggccccttgcagcagaagcaccagcgaatctacagccgccctgggctgcctcgtgaaggactactttcccgagcccgtgaccgtgtcctggaactctggcgctctgacaagcggcgtgcacacctttccagccgtgctccagagcagcggcctgtactctctgagcagcgtcgtgacagtgcccagcagcagcctgggcaccaagacctacacctgtaacgtggaccacaagcccagcaacaccaaggtggacaagcgggtggaatctaagtacggccctccctgccctccttgcccagcccctgaatttctgggcggaccctccgtgttcctgttccccccaaagcccaaggacaccctgatgatcagccggacccccgaagtgacctgcgtggtggtggatgtgtcccaggaagatcccgaggtgcagttcaattggtacgtggacggcgtggaagtgcacaacgccaagaccaagcccagagaggaacagttcaacagcacctaccgggtggtgtccgtgctgaccgtgctgcaccaggactggctgaacggcaaagagtacaagtgcaaggtgtccaacaagggcctgcccagctccatcgagaaaaccatcagcaaggccaagggccagccccgcgagcctcaagtgtgtaccctgccccctagccaggaagagatgaccaagaaccaggtgtccctgagctgtgccgtgaaaggcttctaccccagcgacattgccgtggaatgggagagcaacggccagcccgagaacaactacaagaccaccccccctgtgctggacagcgacggctcattcttcctggtgtccaagctgaccgtggacaagagccggtggcaggaaggcaacgtgttcagctgctccgtgatgcacgaggccctgcacaaccactacacccagaagtccctgtctctgtccctgggcaag

SEQ ID NO: 12 - DNA, 1026 bp, synthetic construct
  misc_feature 1..1026: note = Synthetic Construct
  source 1..1026: mol_type = other DNA
gacatcgtgatgacccagacccccctgagcctgagcgtgacacctggacagcctgccagcatcagctgcaagagcagccagagcctggtgcacaacaacgccaacacctacctgagctggtatctgcagaagcccggccagagcccccagtccctgatctacaaggtgtccaacagattcagcggcgtgcccgacagattctccggcagcggctctggcaccgacttcaccctgaagatcagccgggtggaagccgaggacgtgggcgtgtactattgtggccagggcacccagtaccccttcacctttggcagcggcaccaaggtggaaatcaagggccagcccaaggccgcccccgacatcgtgctgacacagagccctgctagcctggccgtgtctcctggacagagggccaccatcacctgtagagccagcgagagcgtggaatattacgtgaccagcctgatgcagtggtatcagcagaagcccggccagccccccaagctgctgattttcgccgccagcaacgtggaaagcggcgtgccagccagattttccggcagcggctctggcaccgacttcaccctgaccatcaaccccgtggaagccaacgacgtggccaactactactgccagcagagccggaaggtgccctacacctttggccagggcaccaagctggaaatcaagaccaagggccccagccgtacggtggccgctcccagcgtgttcatcttcccacctagcgacgagcagctgaagtccggcacagcctctgtcgtgtgcctgctgaacaacttctacccccgcgaggccaaagtgcagtggaaggtggacaacgccctgcagagcggcaacagccaggaaagcgtgaccgagcaggacagcaaggactccacctacagcctgagcagcaccctgacactgagcaaggccgactacgagaagcacaaggtgtacgcctgcgaagtgacccaccagggcctgtctagccccgtgaccaagagcttcaaccggggcgagtgt

SEQ ID NO: 13 - protein, 451 aa, synthetic construct
  REGION 1..451: note = Synthetic Construct
QVQLVQSGAEVKKPGSSVKVSCKASGYAFSSYWMNWVRQAPGQGLEWIGQIWPGDGDTNYNQKFKGRATLTADESTSTAYMELSSLRSEDTAVYYCARRETTTVGRYYYAMDYWGQGTTVTVSSASTKGPSVFPLAPCSRSTSESTAALGCLVKDYFPEPVTVSWNSGALTSGVHTFPAVLQSSGLYSLSSVVTVPSSSLGTKTYTCNVDHKPSNTKVDKRVESKYGPPCPPCPAPEFLGGPSVFLFPPKPKDTLMISRTPEVTCVVVDVSQEDPEVQFNWYVDGVEVHNAKTKPREEQFNSTYRVVSVLTVLHQDWLNGKEYKCKVSNKGLPSSIEKTISKAKGQPREPQVYTLPPCQEEMTKNQVSLWCLVKGFYPSDIAVEWESNGQPENNYKTTPPVLDSDGSFFLYSKLTVDKSRWQEGNVFSCSVMHEALHNHYTQKSLSLSLGK

SEQ ID NO: 14 - protein, 218 aa, synthetic construct
  REGION 1..218: note = Synthetic Construct
DLVLTQSPASLAVSPGQRATITCKASQSVDYDGDSYLNWYQQKPGQPPKLLIYDASNLVSGVPARFSGSGSGTDFTLTINPVEANDTANYYCQQSTEDPWTFGQGTKLEIKRTVAAPSVFIFPPSDEQLKSGTASVVCLLNNFYPREAKVQWKVDNALQSGNSQESVTEQDSKDSTYSLSSTLTLSKADYEKHKVYACEVTHQGLSSPVTKSFNRGEC

SEQ ID NO: 15 - DNA, 1353 bp, synthetic construct
  misc_feature 1..1353: note = Synthetic Construct
  source 1..1353: mol_type = other DNA
caggtgcagctggtgcagagcggcgccgaagtgaagaagcctggcagcagcgtgaaggtgagctgcaaggccagcggctatgccttcagcagctactggatgaactgggtgaggcaggcacctggccagggcctggagtggataggccaaatatggcctggcgatggcgacaccaactacaaccagaagttcaagggcagagcgaccttgaccgccgacgagagcaccagcaccgcgtacatggagctgagcagcctgaggagcgaggacaccgccgtgtactattgcgccagaagggagaccaccaccgtgggcaggtactactacgccatggactactggggccagggaaccaccgtgaccgtgagcagcgcctcgaccaagggcccatcggtgttccctctggccccttgcagcagaagcaccagcgaatctacagccgccctgggctgcctcgtgaaggactactttcccgagcccgtgaccgtgtcctggaactctggcgctctgacaagcggcgtgcacacctttccagccgtgctccagagcagcggcctgtactctctgagcagcgtcgtgacagtgcccagcagcagcctgggcaccaagacctacacctgtaacgtggaccacaagcccagcaacaccaaggtggacaagcgggtggaatctaagtacggccctccctgccctccttgcccagcccctgaatttctgggcggaccctccgtgttcctgttccccccaaagcccaaggacaccctgatgatcagccggacccccgaagtgacctgcgtggtggtggatgtgtcccaggaagatcccgaggtgcagttcaattggtacgtggacggcgtggaagtgcacaacgccaagaccaagcccagagaggaacagttcaacagcacctaccgggtggtgtccgtgctgaccgtgctgcaccaggactggctgaacggcaaagagtacaagtgcaaggtgtccaacaagggcctgcccagctccatcgagaaaaccatcagcaaggccaagggccagccccgcgagcctcaagtgtataccctgcccccttgccaggaagagatgaccaagaaccaggtgtccctgtggtgtctcgtgaaaggcttctaccccagcgacattgccgtggaatgggagagcaacggccagcccgagaacaactacaagaccaccccccctgtgctggacagcgacggctcattcttcctgtactccaagctgaccgtggacaagagccggtggcaggaaggcaacgtgttcagctgctccgtgatgcacgaggccctgcacaaccactacacccagaagtccctgtctctgtccctgggcaag

SEQ ID NO: 16 - DNA, 654 bp, synthetic construct
  misc_feature 1..654: note = Synthetic Construct
  source 1..654: mol_type = other DNA
gacctcgtgctgacccagagccctgcgagcctggctgtgagccctggccagagagccaccatcacctgcaaagccagccagagcgtggactacgacggcgacagctacctcaactggtaccagcagaagcctggccagccccccaagctgctgatttacgatgccagcaacctggtgagcggcgtgcctgctagattcagcggctccggcagcggcaccgacttcaccctgaccatcaaccccgtggaggccaacgacaccgccaactactactgccagcagagcacggaggacccctggaccttcggccagggcacaaagctggagatcaagcgtacggtggccgctcccagcgtgttcatcttcccacctagcgacgagcagctgaagtccggcacagcctctgtcgtgtgcctgctgaacaacttctacccccgcgaggccaaagtgcagtggaaggtggacaacgccctgcagagcggcaacagccaggaaagcgtgaccgagcaggacagcaaggactccacctacagcctgagcagcaccctgacactgagcaaggccgactacgagaagcacaaggtgtacgcctgcgaagtgacccaccagggcctgtctagccccgtgaccaagagcttcaaccggggcgagtgt

SEQ ID NO: 17 - protein, 447 aa, synthetic construct
  REGION 1..447: note = Synthetic Construct
QVQLVQSGAEVAKPGTSVKLSCKASGYTFTDYWMQWVKQRPGQGLEWIGTIYPGDGDTGYAQKFQGKATLTADKSSKTVYMHLSSLASEDSAVYYCARGDYYGSNSLDYWGQGTSVTVSSASTKGPSVFPLAPCSRSTSESTAALGCLVKDYFPEPVTVSWNSGALTSGVHTFPAVLQSSGLYSLSSVVTVPSSSLGTKTYTCNVDHKPSNTKVDKRVESKYGPPCPPCPAPEFLGGPSVFLFPPKPKDTLMISRTPEVTCVVVDVSQEDPEVQFNWYVDGVEVHNAKTKPREEQFNSTYRVVSVLTVLHQDWLNGKEYKCKVSNKGLPSSIEKTISKAKGQPREPQVYTLPPCQEEMTKNQVSLWCLVKGFYPSDIAVEWESNGQPENNYKTTPPVLDSDGSFFLYSKLTVDKSRWQEGNVFSCSVMHEALHNHYTQKSLSLSLGK

SEQ ID NO: 18 - protein, 214 aa, synthetic construct
  REGION 1..214: note = Synthetic Construct
DIVMTQSHLSMSTSLGDPVSITCKASQDVSTVVAWYQQKPGQSPRRLIYSASYRYIGVPDRFTGSGAGTDFTFTISSVQAEDLAVYYCQQHYSPPYTFGGGTKLEIKRTVAAPSVFIFPPSDEQLKSGTASVVCLLNNFYPREAKVQWKVDNALQSGNSQESVTEQDSKDSTYSLSSTLTLSKADYEKHKVYACEVTHQGLSSPVTKSFNRGEC

SEQ ID NO: 19 - DNA, 1341 bp, synthetic construct
  misc_feature 1..1341: note = Synthetic Construct
  source 1..1341: mol_type = other DNA
caggtgcagctggtgcagtctggcgccgaagtggccaagcctggcacaagcgtgaagctgagctgcaaggccagcggctacaccttcaccgactactggatgcagtgggtcaagcagaggccaggccagggcctggaatggatcggcacaatctatcccggcgacggcgataccggctacgcccagaagtttcagggcaaggccaccctgaccgccgacaagagcagcaagaccgtgtacatgcacctgagcagcctggccagcgaggacagcgccgtgtactattgcgccagaggcgactactacggcagcaacagcctggactattggggccagggcaccagcgtgacagtgtctagtgcgtcgaccaagggcccatcggtgttccctctggccccttgcagcagaagcaccagcgaatctacagccgccctgggctgcctcgtgaaggactactttcccgagcccgtgaccgtgtcctggaactctggcgctctgacaagcggcgtgcacacctttccagccgtgctccagagcagcggcctgtactctctgagcagcgtcgtgacagtgcccagcagcagcctgggcaccaagacctacacctgtaacgtggaccacaagcccagcaacaccaaggtggacaagcgggtggaatctaagtacggccctccctgccctccttgcccagcccctgaatttctgggcggaccctccgtgttcctgttccccccaaagcccaaggacaccctgatgatcagccggacccccgaagtgacctgcgtggtggtggatgtgtcccaggaagatcccgaggtgcagttcaattggtacgtggacggcgtggaagtgcacaacgccaagaccaagcccagagaggaacagttcaacagcacctaccgggtggtgtccgtgctgaccgtgctgcaccaggactggctgaacggcaaagagtacaagtgcaaggtgtccaacaagggcctgcccagctccatcgagaaaaccatcagcaaggccaagggccagccccgcgagcctcaagtgtataccctgcccccttgccaggaagagatgaccaagaaccaggtgtccctgtggtgtctcgtgaaaggcttctaccccagcgacattgccgtggaatgggagagcaacggccagcccgagaacaactacaagaccaccccccctgtgctggacagcgacggctcattcttcctgtactccaagctgaccgtggacaagagccggtggcaggaaggcaacgtgttcagctgctccgtgatgcacgaggccctgcacaaccactacacccagaagtccctgtctctgtccctgggcaag

SEQ ID NO: 20 - DNA, 642 bp, synthetic construct
  misc_feature 1..642: note = Synthetic Construct
  source 1..642: mol_type = other DNA
gacatcgtgatgacccagagccacctgagcatgagcaccagcctgggcgaccccgtgtccatcacctgtaaagccagccaggacgtgtccaccgtggtggcctggtatcagcagaagcctggccagagccccagacggctgatctacagcgccagctatcggtacatcggcgtgcccgacagattcaccggaagcggagccggcaccgacttcaccttcaccatcagctctgtgcaggccgaggacctggccgtgtactactgccagcagcactacagccccccctacacctttggcggaggcaccaagctggaaatcaagcgtacggtggccgctcccagcgtgttcatcttcccacctagcgacgagcagctgaagtccggcacagcctctgtcgtgtgcctgctgaacaacttctacccccgcgaggccaaagtgcagtggaaggtggacaacgccctgcagagcggcaacagccaggaaagcgtgaccgagcaggacagcaaggactccacctacagcctgagcagcaccctgacactgagcaaggccgactacgagaagcacaaggtgtacgcctgcgaagtgacccaccagggcctgtctagccccgtgaccaagagcttcaaccggggcgagtgt

SEQ ID NO: 21 - protein, 445 aa, synthetic construct
  REGION 1..445: note = Synthetic Construct
QVQLVQSGAEVKKPGSSVKVSCKASGYIFTNYNIHWVKKSPGQGLEWIGAIYPGNGDAPYSQKFQGKATLTADTSTSTTYMELSSLRSEDTAVYYCVRANWDVAFAYWGQGTLVTVSSASTKGPSVFPLAPCSRSTSESTAALGCLVKDYFPEPVTVSWNSGALTSGVHTFPAVLQSSGLYSLSSVVTVPSSSLGTKTYTCNVDHKPSNTKVDKRVESKYGPPCPPCPAPEFLGGPSVFLFPPKPKDTLMISRTPEVTCVVVDVSQEDPEVQFNWYVDGVEVHNAKTKPREEQFNSTYRVVSVLTVLHQDWLNGKEYKCKVSNKGLPSSIEKTISKAKGQPREPQVYTLPPCQEEMTKNQVSLWCLVKGFYPSDIAVEWESNGQPENNYKTTPPVLDSDGSFFLYSKLTVDKSRWQEGNVFSCSVMHEALHNHYTQKSLSLSLGK

SEQ ID NO: 22 - protein, 213 aa, synthetic construct
  REGION 1..213: note = Synthetic Construct
DIQMTQSPSSLSASVGDRVTITCKASQDIDRYMAWYQDKPGKAPRLLIHDTSTLQSGVPSRFSGSGSGRDYTLTISNLEPEDFATYYCLQYDNLWTFGGGTKVEIKRTVAAPSVFIFPPSDEQLKSGTASVVCLLNNFYPREAKVQWKVDNALQSGNSQESVTEQDSKDSTYSLSSTLTLSKADYEKHKVYACEVTHQGLSSPVTKSFNRGEC

SEQ ID NO: 23 - DNA, 1335 bp, synthetic construct
  misc_feature 1..1335: note = Synthetic Construct
  source 1..1335: mol_type = other DNA
caggtgcagctggtgcagtctggcgccgaagtgaagaaacccggcagcagcgtgaaggtgtcctgcaaggccagcggctacatcttcaccaactacaacatccactgggtcaagaagtccccaggccagggcctggaatggatcggcgccatctatcccggaaacggcgacgccccttacagccagaagttccagggcaaggccaccctgaccgccgataccagcacctccaccacctacatggaactgagcagcctgcggagcgaggacaccgccgtgtactattgcgtgcgggccaactgggatgtggccttcgcctattggggccagggcacactcgtgaccgtgtcctctgcgtcgaccaagggcccatcggtgttccctctggccccttgcagcagaagcaccagcgaatctacagccgccctgggctgcctcgtgaaggactactttcccgagcccgtgaccgtgtcctggaactctggcgctctgacaagcggcgtgcacacctttccagccgtgctccagagcagcggcctgtactctctgagcagcgtcgtgacagtgcccagcagcagcctgggcaccaagacctacacctgtaacgtggaccacaagcccagcaacaccaaggtggacaagcgggtggaatctaagtacggccctccctgccctccttgcccagcccctgaatttctgggcggaccctccgtgttcctgttccccccaaagcccaaggacaccctgatgatcagccggacccccgaagtgacctgcgtggtggtggatgtgtcccaggaagatcccgaggtgcagttcaattggtacgtggacggcgtggaagtgcacaacgccaagaccaagcccagagaggaacagttcaacagcacctaccgggtggtgtccgtgctgaccgtgctgcaccaggactggctgaacggcaaagagtacaagtgcaaggtgtccaacaagggcctgcccagctccatcgagaaaaccatcagcaaggccaagggccagccccgcgagcctcaagtgtataccctgcccccttgccaggaagagatgaccaagaaccaggtgtccctgtggtgtctcgtgaaaggcttctaccccagcgacattgccgtggaatgggagagcaacggccagcccgagaacaactacaagaccaccccccctgtgctggacagcgacggctcattcttcctgtactccaagctgaccgtggacaagagccggtggcaggaaggcaacgtgttcagctgctccgtgatgcacgaggccctgcacaaccactacacccagaagtccctgtctctgtccctgggcaag

SEQ ID NO: 24 - DNA, 639 bp, synthetic construct
  misc_feature 1..639: note = Synthetic Construct
  source 1..639: mol_type = other DNA
gacatccagatgacccagagccccagcagcctgtctgccagcgtgggcgacagagtgaccatcacatgcaaggccagccaggacatcgatcggtacatggcctggtatcaggacaagcccggcaaggcccccagactgctgatccacgataccagcacactgcagagcggcgtgcccagcagattttccggctctggcagcggcagagactacaccctgaccatcagcaacctggaacccgaggacttcgccacctactactgcctgcagtacgacaacctgtggaccttcggcggaggcaccaaggtggaaatcaagcgtacggtggccgctcccagcgtgttcatcttcccacctagcgacgagcagctgaagtccggcacagcctctgtcgtgtgcctgctgaacaacttctacccccgcgaggccaaagtgcagtggaaggtggacaacgccctgcagagcggcaacagccaggaaagcgtgaccgagcaggacagcaaggactccacctacagcctgagcagcaccctgacactgagcaaggccgactacgagaagcacaaggtgtacgcctgcgaagtgacccaccagggcctgtctagccccgtgaccaagagcttcaaccggggcgagtgt

SEQ ID NO: 25 - protein, 8 aa, synthetic construct
  REGION 1..8: note = Synthetic Construct
GFNIKDTY

SEQ ID NO: 26 - protein, 8 aa, synthetic construct
  REGION 1..8: note = Synthetic Construct
IYPTNGYT

SEQ ID NO: 27 - protein, 13 aa, synthetic construct
  REGION 1..13: note = Synthetic Construct
SRWGGDGFYAMDY

SEQ ID NO: 28 - protein, 8 aa, synthetic construct
  REGION 1..8: note = Synthetic Construct
GYTFTSYY

SEQ ID NO: 29 - protein, 8 aa, synthetic construct
  REGION 1..8: note = Synthetic Construct
IYPGNVNT

SEQ ID NO: 30 - protein, 13 aa, synthetic construct
  REGION 1..13: note = Synthetic Construct
TRSHYGLDWNFDV

SEQ ID NO: 31 - protein, 8 aa, synthetic construct
  REGION 1..8: note = Synthetic Construct
GFSLSDYG

SEQ ID NO: 32 - protein, 7 aa, synthetic construct
  REGION 1..7: note = Synthetic Construct
IWAGGGT

SEQ ID NO: 33 - protein, 13 aa, synthetic construct
  REGION 1..13: note = Synthetic Construct
ARDKGYSYYYSMD

SEQ ID NO: 34 - protein, 8 aa, synthetic construct
  REGION 1..8: note = Synthetic Construct
GFTFTKAW

SEQ ID NO: 35 - protein, 7 aa, synthetic construct
  REGION 1..7: note = Synthetic Construct
IKDKSNS

SEQ ID NO: 36 - protein, 12 aa, synthetic construct
  REGION 1..12: note = Synthetic Construct
RGVYYALSPFDY

SEQ ID NO: 37 - protein, 8 aa, synthetic construct
  REGION 1..8: note = Synthetic Construct
GYAFSSYW

SEQ ID NO: 38 - protein, 8 aa, synthetic construct
  REGION 1..8: note = Synthetic Construct
IWPGDGDT

SEQ ID NO: 39 - protein, 16 aa, synthetic construct
  REGION 1..16: note = Synthetic Construct
ARRETTTVGRYYYAMD

SEQ ID NO: 40 - protein, 8 aa, synthetic construct
  REGION 1..8: note = Synthetic Construct
GYTFTDYW

SEQ ID NO: 41 - protein, 8 aa, synthetic construct
  REGION 1..8: note = Synthetic Construct
IYPGDGDT

SEQ ID NO: 42 - protein, 13 aa, synthetic construct
  REGION 1..13: note = Synthetic Construct
ARGDYYGSNSLDY

SEQ ID NO: 43 - protein, 6 aa, synthetic construct
  REGION 1..6: note = Synthetic Construct
QDVNTA

SEQ ID NO: 44 - skipped

SEQ ID NO: 45 - protein, 9 aa, synthetic construct
  REGION 1..9: note = Synthetic Construct
QQHYTTPPT

SEQ ID NO: 46 - protein, 6 aa, synthetic construct
  REGION 1..6: note = Synthetic Construct
QNIYVW

SEQ ID NO: 47 - skipped

SEQ ID NO: 48 - protein, 9 aa, synthetic construct
  REGION 1..9: note = Synthetic Construct
QQGQTYPYT

SEQ ID NO: 49 - protein, 10 aa, synthetic construct
  REGION 1..10: note = Synthetic Construct
ESVEYYVTSL

SEQ ID NO: 50 - skipped

SEQ ID NO: 51 - protein, 9 aa, synthetic construct
  REGION 1..9: note = Synthetic Construct
QQSRKVPYT

SEQ ID NO: 52 - protein, 11 aa, synthetic construct
  REGION 1..11: note = Synthetic Construct
QSLVHNNANTY

SEQ ID NO: 53 - skipped

SEQ ID NO: 54 - protein, 7 aa, synthetic construct
  REGION 1..7: note = Synthetic Construct
GQGTQYP

SEQ ID NO: 55 - protein, 10 aa, synthetic construct
  REGION 1..10: note = Synthetic Construct
QSVDYDGDSY

SEQ ID NO: 56 - skipped

SEQ ID NO: 57 - protein, 9 aa, synthetic construct
  REGION 1..9: note = Synthetic Construct
QQSTEDPWT

SEQ ID NO: 58 - protein, 6 aa, synthetic construct
  REGION 1..6: note = Synthetic Construct
QDVSTV

SEQ ID NO: 59 - protein, 9 aa, synthetic construct
  REGION 1..9: note = Synthetic Construct
QQHYSPPYT

SEQ ID NO: 60 - protein, 450 aa, synthetic construct
  REGION 1..450: note = Synthetic Construct
EVQLVESGGGLVQPGRSLRLSCAASGFTFDDYAMHWVRQAPGKGLEWVSAITWNSGHIDYADSVEGRFTISRDNAKNSLYLQMNSLRAEDTAVYYCAKVSYLSTASSLDYWGQGTLVTVSSASTKGPSVFPLAPSSKSTSGGTAALGCLVKDYFPEPVTVSWNSGALTSGVHTFPAVLQSSGLYSLSSVVTVPSSSLGTQTYICNVNHKPSNTKVDKKVEPKSCDKTHTCPPCPAPELLGGPSVFLFPPKPKDTLMISRTPEVTCVVVDVSHEDPEVKFNWYVDGVEVHNAKTKPREEQYNSTYRVVSVLTVLHQDWLNGKEYKCKVSNKALPAPIEKTISKAKGQPREPQVCTLPPSRDELTKNQVSLSCAVKGFYPSDIAVEWESNGQPENNYKTTPPVLDSDGSFFLVSKLTVDKSRWQQGNVFSCSVMHEALHNHYTQKSLSLSPG

SEQ ID NO: 61 - protein, 213 aa, synthetic construct
  REGION 1..213: note = Synthetic Construct
DIQMTQSPSSLSASVGDRVTITCRASQGIRNYLAWYQQKPGKAPKLLIYAASTLQSGVPSRFSGSGSGTDFTLTISSLQPEDVATYYCQRYNRAPYTFGQGTKVEIKGQPKAAPSVTLFPPSSEELQANKATLVCLISDFYPGAVTVAWKADSSPVKAGVETTTPSKQSNNKYAASSYLSLTPEQWKSHRSYSCQVTHEGSTVEKTVAPTECS

SEQ ID NO: 62 - protein, 570 aa, synthetic construct
  REGION 1..570: note = Synthetic Construct
QVQLQQSGPELVKPGASVKISCKASGYSFTSYWIHWIKQRPGQGLEWIGMIDPSDGETRLNQRFQGRATLTVDESTSTAYMQLRSPTSEDSAVYYCTRLKEYGNYDSFYFDVWGAGTLVTVSSEVQLKESGPGLVAPGGSLSITCTVSGFSLTDSSINWVRQPPGKGLEWLGMIWGDGRIDYADALKSRLSISKDSSKSQVFLEMTSLRTDDTATYYCARDGYFPYAMDFWGQGTSVTVSSASTKGPSVFPLAPSSKSTSGGTAALGCLVKDYFPEPVTVSWNSGALTSGVHTFPAVLQSSGLYSLSSVVTVPSSSLGTQTYICNVNHKPSNTKVDKKVEPKSCDKTHTCPPCPAPELLGGPSVFLFPPKPKDTLMISRTPEVTCVVVDVSHEDPEVKFNWYVDGVEVHNAKTKPREEQYNSTYRVVSVLTVLHQDWLNGKEYKCKVSNKALPAPIEKTISKAKGQPREPQVYTLPPCRDELTKNQVSLWCLVKGFYPSDIAVEWESNGQPENNYKTTPPVLDSDGSFFLYSKLTVDKSRWQQGNVFSCSVMHEALHNRFTQKSLSLSPG

SEQ ID NO: 63 - protein, 345 aa, synthetic construct
  REGION 1..345: note = Synthetic Construct
DIVLTQSPASLAVSLGQRATISCRASESVDSYGQSYMHWYQQKAGQPPKLLIYLASNLESGVPARFSGSGSRTDFTLTIDPVQAEDAATYYCQQNAEDSRTFGGGTKLEIKGGSGSSGSGGDIQMTQSPASLSVSVGDTITLTCHASQNIDVWLSWFQQKPGNIPKLLIYKASNLHTGVPSRFSGSGSGTGFTLTISSLQPEDIATYYCQQAHSYPFTFGGGTKLEIKGGSGSSGSGGRTVAAPSVFIFPPSDEQLKSGTASVVCLLNNFYPREAKVQWKVDNALQSGNSQESVTEQDSKDSTYSLSSTLTLSKADYEKHKVYACEVTHQGLSSPVTKSFNRGEC

SEQ ID NO: 64 - DNA, 1350 bp, synthetic construct
  misc_feature 1..1350: note = Synthetic Construct
  source 1..1350: mol_type = other DNA
gaggtgcagctggtggaaagcggcggaggactggtgcagcccggcagaagcctgagactgagctgcgccgccagcggcttcaccttcgacgactacgccatgcactgggtccgccaggcccctggcaagggcctggaatgggtgtccgccatcacctggaacagcggccacatcgactacgccgacagcgtggaaggccggttcaccatcagccgggacaacgccaagaacagcctgtacctgcagatgaacagcctgcgggccgaggacaccgccgtgtactactgcgccaaggtgtcctacctgagcaccgccagcagcctggactactggggccagggcaccctggtgacagtgtccagcgcttccaccaagggccccagcgtgttccccctggcccctagcagcaagagcacatctggcggcacagccgccctgggctgcctggtcaaggactacttccccgagcccgtgacagtgtcctggaactctggcgccctgaccagcggagtgcataccttccctgccgtgctgcagtccagcggcctgtacagcctgagcagcgtggtcacagtgcccagcagcagcctgggcacccagacctacatctgcaacgtgaaccacaagcccagcaacaccaaggtggacaagaaggtggaacccaagagctgcgacaagacccacacctgtcccccctgccctgcccctgaactgctgggcggaccctccgtgttcctgttccccccaaagcccaaggacaccctgatgatcagccggacccccgaagtgacctgcgtggtggtggacgtgtcccacgaggaccctgaagtgaagttcaattggtacgtggacggcgtggaagtgcataacgccaagaccaagcccagagaggaacagtacaacagcacctaccgggtggtgtccgtgctgaccgtgctgcaccaggactggctgaacggcaaagagtacaagtgcaaggtgtccaacaaggccctgcctgcccccatcgagaaaaccatcagcaaggccaagggccagcctagagagccccaagtctgcaccctgccccccagcagagatgagctgaccaagaaccaggtgtccctgagctgcgccgtgaagggcttctaccccagcgatatcgccgtggaatgggagagcaacggccagcccgagaacaactacaagaccaccccccctgtgctggacagcgacggctcattcttcctggtgtccaagctgacagtggacaagagccggtggcagcagggcaacgtgttcagctgcagcgtgatgcacgaggccctgcacaaccattacacccagaagtccctgagcctgagccccggc

SEQ ID NO: 65 - DNA, 639 bp, synthetic construct
  misc_feature 1..639: note = Synthetic Construct
  source 1..639: mol_type = other DNA
gacatccagatgacccagagccccagcagcctgagcgccagcgtgggcgacagagtgaccatcacctgtcgggccagccagggcatccggaactacctggcctggtatcagcagaagcccggcaaggcccccaagctgctgatctacgccgccagcacactgcagagcggcgtgcccagcagattcagcggcagcggctccggcaccgacttcaccctgaccatcagcagcctgcagcccgaggacgtggccacctactactgccagcggtacaacagagccccctacaccttcggccagggcaccaaggtggaaatcaagggacagcccaaggctgccccctcggtcaccctgttccccccaagcagcgaggaactgcaggccaacaaggccaccctcgtgtgcctgatcagcgacttctaccctggcgccgtgaccgtggcctggaaggccgatagctctcccgtgaaggccggcgtggaaaccaccacccccagcaagcagagcaacaacaaatacgccgcctccagctacctgagcctgacccccgagcagtggaagtcccaccggtcctacagctgccaggtcacacacgagggcagcaccgtggaaaagaccgtggcccccaccgagtgcagc

SEQ ID NO: 66 - DNA, 1710 bp, synthetic construct
  misc_feature 1..1710: note = Synthetic Construct
  source 1..1710: mol_type = other DNA
caggtgcagctgcagcagagcggccctgagctggtcaagcctggcgccagcgtgaagatcagctgcaaggccagcggctacagcttcaccagctactggatccactggatcaagcagcggcctggccagggcctggaatggatcggcatgatcgaccccagcgacggcgagacacggctgaaccagagattccagggcagagccaccctgaccgtggacgagagcaccagcaccgcctacatgcagctgcggagccccaccagcgaggacagcgccgtgtactactgcacccggctgaaagagtacggcaactacgacagcttctacttcgacgtgtggggagccggcaccctggtcaccgtgtccagcgaagtgcagctgaaagaaagcggccctggcctggtggcccctggcggcagcctgagcatcacctgtaccgtgtccggcttcagcctgaccgacagcagcatcaactgggtccgacagccccctggcaagggcctcgagtggctgggaatgatctggggcgacggccggatcgactacgccgacgccctgaagtcccggctgagcatcagcaaggacagcagcaagagccaggtgttcctggaaatgaccagcctgcggaccgacgacaccgccacctactactgcgccagggacggctacttcccctacgccatggatttctggggccagggcaccagcgtgaccgtgtcctctgcttccaccaagggccccagcgtgttccctctggcccctagcagcaagagcacatctggcggaacagccgccctgggctgcctggtcaaggactactttcccgagcccgtgaccgtgtcctggaactctggtgccctgacaagcggagtgcataccttccctgccgtgctgcagagcagcggcctgtactctctgagcagcgtggtcaccgtgccaagcagcagcctgggcacccagacctacatctgcaacgtgaaccacaagccctccaacaccaaggtggacaagaaggtggaacccaagagctgcgacaagacccacacctgtcctccctgtcctgcccctgaactgctgggcggaccctccgtgttcctgttccctccaaagcccaaggataccctgatgatcagccggacccctgaagtgacctgcgtggtggtggacgtgtcccacgaggatcccgaagtgaagttcaattggtacgtggacggcgtggaagtgcataacgccaagaccaagcccagagaggaacagtacaacagcacctaccgggtggtgtccgtgctgacagtgctgcaccaggactggctgaacggcaaagagtacaagtgcaaggtgtccaacaaggccctgccagcccctatcgagaaaaccatcagcaaggccaagggccagccccgcgagcctcaggtgtacacactgcctccatgccgggacgagctgaccaagaaccaggtgtccctgtggtgcctcgtgaagggcttctacccctccgatatcgccgtggaatgggagagcaacggccagcccgagaacaactacaagaccacccctcccgtgctggacagcgacggctcattcttcctgtacagcaagctgaccgtggacaagtcccggtggcagcagggcaacgtgttcagctgctctgtgatgcacgaggccctgcacaaccggttcacccagaagtccctgagcctgagccctggc

SEQ ID NO: 67 - DNA, 1035 bp, synthetic construct
  misc_feature 1..1035: note = Synthetic Construct
  source 1..1035: mol_type = other DNA
gacatcgtgctgacccagagccctgccagcctggccgtgtctctgggccagagagccaccatcagctgccgggccagcgagagcgtggacagctacggccagagctacatgcactggtatcagcagaaggccggccagccccccaagctgctgatctacctggccagcaacctggaaagcggcgtgcccgccagattcagcggcagcggcagcagaaccgacttcaccctgaccatcgaccccgtgcaggccgaggacgccgccacctactactgccagcagaacgccgaggacagccggaccttcggcggaggcaccaagctggaaatcaagggcggctccggcagcagcggctctggcggcgatatccagatgacccagtcccccgcctccctgagcgtgtccgtgggcgacaccatcaccctgacatgccacgccagccagaacatcgacgtgtggctgagctggttccagcagaagcctggcaacatccctaagctgctcatctataaggcctccaacctgcacaccggcgtgcccagcaggttttccggctctggcagcggcaccggctttaccctgacaatcagcagcctgcagcccgaggatatcgccacatattactgtcagcaggcccacagctaccccttcacctttggcggcggaacaaagctcgagattaagggcggcagcggaagctccggctccggcggacgtacggtggccgctccttccgtgttcatcttccctccctccgacgagcagctgaagtccggcaccgcctccgtggtgtgtctgctgaacaacttctaccctcgggaggccaaggtgcagtggaaggtggacaacgccctgcagtccggcaactcccaggagtccgtcaccgagcaggactccaaggacagcacctactccctgtcctccaccctgaccctgtccaaggccgactacgagaagcacaaggtgtacgcctgtgaggtgacccaccagggcctgtccagccctgtgaccaagtccttcaaccggggcgagtgc

SEQ ID NO: 68 - protein, 570 aa, synthetic construct
  REGION 1..570: note = Synthetic Construct
EVQLKESGPGLVAPGGSLSITCTVSGFSLTDSSINWVRQPPGKGLEWLGMIWGDGRIDYADALKSRLSISKDSSKSQVFLEMTSLRTDDTATYYCARDGYFPYAMDFWGQGTSVTVSSQVQLQQSGPELVKPGASVKISCKASGYSFTSYWIHWIKQRPGQGLEWIGMIDPSDGETRLNQRFQGRATLTVDESTSTAYMQLRSPTSEDSAVYYCTRLKEYGNYDSFYFDVWGAGTLVTVSSASTKGPSVFPLAPSSKSTSGGTAALGCLVKDYFPEPVTVSWNSGALTSGVHTFPAVLQSSGLYSLSSVVTVPSSSLGTQTYICNVNHKPSNTKVDKKVEPKSCDKTHTCPPCPAPELLGGPSVFLFPPKPKDTLMISRTPEVTCVVVDVSHEDPEVKFNWYVDGVEVHNAKTKPREEQYNSTYRVVSVLTVLHQDWLNGKEYKCKVSNKALPAPIEKTISKAKGQPREPQVYTLPPCRDELTKNQVSLWCLVKGFYPSDIAVEWESNGQPENNYKTTPPVLDSDGSFFLYSKLTVDKSRWQQGNVFSCSVMHEALHNRFTQKSLSLSPG

SEQ ID NO: 69 - protein, 345 aa, synthetic construct
  REGION 1..345: note = Synthetic Construct
DIQMTQSPASLSVSVGDTITLTCHASQNIDVWLSWFQQKPGNIPKLLIYKASNLHTGVPSRFSGSGSGTGFTLTISSLQPEDIATYYCQQAHSYPFTFGGGTKLEIKGGSGSSGSGGDIVLTQSPASLAVSLGQRATISCRASESVDSYGQSYMHWYQQKAGQPPKLLIYLASNLESGVPARFSGSGSRTDFTLTIDPVQAEDAATYYCQQNAEDSRTFGGGTKLEIKGGSGSSGSGGRTVAAPSVFIFPPSDEQLKSGTASVVCLLNNFYPREAKVQWKVDNALQSGNSQESVTEQDSKDSTYSLSSTLTLSKADYEKHKVYACEVTHQGLSSPVTKSFNRGEC

SEQ ID NO: 70 - DNA, 1035 bp, synthetic construct
  misc_feature 1..1035: note = Synthetic Construct
  source 1..1035: mol_type = other DNA
gacatccagatgacccagagccccgccagcctgagcgtgtccgtgggcgataccatcaccctgacctgccacgccagccagaacatcgacgtgtggctgagctggttccagcagaagcccggcaacatccccaagctgctgatctacaaggccagcaacctgcacaccggcgtgcccagcagattcagcggctctggcagcggcaccggctttaccctgaccatcagcagcctgcagcccgaggatatcgccacctactactgccagcaggcccacagctaccccttcaccttcggcggaggcaccaagctggaaatcaagggcggcagcggcagctccggctctggcggcgatatcgtgctgacccagtctcccgcctccctggccgtgtctctgggccagagagccaccatcagctgccgggccagcgagagcgtggacagctacggccagagctacatgcactggtatcagcagaaggccggacagccccctaaactgctcatctacctggcctccaacctggaaagcggcgtgcccgccaggttttccggcagcggctccagaaccgacttcaccctgacaatcgaccccgtgcaggccgaggacgccgccacatattactgtcagcagaacgccgaggacagcagaacctttggcggcggaacaaagctcgagattaagggcggctccggctccagcggatctggcggacgtacggtggccgctccttccgtgttcatcttccctccctccgacgagcagctgaagtccggcaccgcctccgtggtgtgtctgctgaacaacttctaccctcgggaggccaaggtgcagtggaaggtggacaacgccctgcagtccggcaactcccaggagtccgtcaccgagcaggactccaaggacagcacctactccctgtcctccaccctgaccctgtccaaggccgactacgagaagcacaaggtgtacgcctgtgaggtgacccaccagggcctgtccagccctgtgaccaagtccttcaaccggggcgagtgc

SEQ ID NO: 71 - protein, 214 aa, synthetic construct
  REGION 1..214: note = Synthetic Construct
DIQMTQSPSSLSASVGDRVTITCRASQGIRNYLAWYQQKPGKAPKLLIYAASTLQSGVPSRFSGSGSGTDFTLTISSLQPEDVATYYCQRYNRAPYTFGQGTKVEIKRTVAAPSVFIFPPSDEQLKSGTASVVCLLNNFYPREAKVQWKVDNALQSGNSQESVTEQDSKDSTYSLSSTLTLSKADYEKHKVYACEVTHQGLSSPVTKSFNRGEC

SEQ ID NO: 72 - DNA, 642 bp, synthetic construct
  misc_feature 1..642: note = Synthetic Construct
  source 1..642: mol_type = other DNA
gacatccagatgacccagagccccagcagcctgagcgccagcgtgggcgacagagtgaccatcacctgtcgggccagccagggcatccggaactacctggcctggtatcagcagaagcccggcaaggcccccaagctgctgatctacgccgccagcacactgcagagcggcgtgcccagcagattcagcggcagcggctccggcaccgacttcaccctgaccatcagcagcctgcagcccgaggacgtggccacctactactgccagcggtacaacagagccccctacaccttcggccagggcaccaaggtggaaatcaagcgtacggtggccgctccttccgtgttcatcttccctccctccgacgagcagctgaagtccggcaccgcctccgtggtgtgtctgctgaacaacttctaccctcgggaggccaaggtgcagtggaaggtggacaacgccctgcagtccggcaactcccaggagtccgtcaccgagcaggactccaaggacagcacctactccctgtcctccaccctgaccctgtccaaggccgactacgagaagcacaaggtgtacgcctgtgaggtgacccaccagggcctgtccagccctgtgaccaagtccttcaaccggggcgagtgc

SEQ ID NO: 73 - protein, 447 aa, synthetic construct
  REGION 1..447: note = Synthetic Construct
EVQLKESGPGLVAPGGSLSITCTVSGFSLTDSSINWVRQPPGKGLEWLGMIWGDGRIDYADALKSRLSISKDSSKSQVFLEMTSLRTDDTATYYCARDGYFPYAMDFWGQGTSVTVSSASTKGPSVFPLAPSSKSTSGGTAALGCLVKDYFPEPVTVSWNSGALTSGVHTFPAVLQSSGLYSLSSVVTVPSSSLGTQTYICNVNHKPSNTKVDKKVEPKSCDKTHTCPPCPAPELLGGPSVFLFPPKPKDTLMISRTPEVTCVVVDVSHEDPEVKFNWYVDGVEVHNAKTKPREEQYNSTYRVVSVLTVLHQDWLNGKEYKCKVSNKALPAPIEKTISKAKGQPREPQVCTLPPSRDELTKNQVSLSCAVKGFYPSDIAVEWESNGQPENNYKTTPPVLDSDGSFFLVSKLTVDKSRWQQGNVFSCSVMHEALHNHYTQKSLSLSPG

SEQ ID NO: 74 - protein, 217 aa, synthetic construct
  REGION 1..217: note = Synthetic Construct
DIVLTQSPASLAVSLGQRATISCRASESVDSYGQSYMHWYQQKAGQPPKLLIYLASNLESGVPARFSGSGSRTDFTLTIDPVQAEDAATYYCQQNAEDSRTFGGGTKLEIKGQPKAAPSVTLFPPSSEELQANKATLVCLISDFYPGAVTVAWKADSSPVKAGVETTTPSKQSNNKYAASSYLSLTPEQWKSHRSYSCQVTHEGSTVEKTVAPTECS

SEQ ID NO: 75 - protein, 573 aa, synthetic construct
  REGION 1..573: note = Synthetic Construct
QVQLQQSGPELVKPGASVKISCKASGYSFTSYWIHWIKQRPGQGLEWIGMIDPSDGETRLNQRFQGRATLTVDESTSTAYMQLRSPTSEDSAVYYCTRLKEYGNYDSFYFDVWGAGTLVTVSSEVQLVESGGGLVQPGRSLRLSCAASGFTFDDYAMHWVRQAPGKGLEWVSAITWNSGHIDYADSVEGRFTISRDNAKNSLYLQMNSLRAEDTAVYYCAKVSYLSTASSLDYWGQGTLVTVSSASTKGPSVFPLAPSSKSTSGGTAALGCLVKDYFPEPVTVSWNSGALTSGVHTFPAVLQSSGLYSLSSVVTVPSSSLGTQTYICNVNHKPSNTKVDKKVEPKSCDKTHTCPPCPAPELLGGPSVFLFPPKPKDTLMISRTPEVTCVVVDVSHEDPEVKFNWYVDGVEVHNAKTKPREEQYNSTYRVVSVLTVLHQDWLNGKEYKCKVSNKALPAPIEKTISKAKGQPREPQVYTLPPCRDELTKNQVSLWCLVKGFYPSDIAVEWESNGQPENNYKTTPPVLDSDGSFFLYSKLTVDKSRWQQGNVFSCSVMHEALHNRFTQKSLSLSPG

SEQ ID NO: 76 - protein, 341 aa, synthetic construct
  REGION 1..341: note = Synthetic Construct
DIQMTQSPSSLSASVGDRVTITCRASQGIRNYLAWYQQKPGKAPKLLIYAASTLQSGVPSRFSGSGSGTDFTLTISSLQPEDVATYYCQRYNRAPYTFGQGTKVEIKGGSGSSGSGGDIQMTQSPASLSVSVGDTITLTCHASQNIDVWLSWFQQKPGNIPKLLIYKASNLHTGVPSRFSGSGSGTGFTLTISSLQPEDIATYYCQQAHSYPFTFGGGTKLEIKGGSGSSGSGGRTVAAPSVFIFPPSDEQLKSGTASVVCLLNNFYPREAKVQWKVDNALQSGNSQESVTEQDSKDSTYSLSSTLTLSKADYEKHKVYACEVTHQGLSSPVTKSFNRGEC

SEQ ID NO: 77 - DNA, 1341 bp, synthetic construct
  misc_feature 1..1341: note = Synthetic Construct
  source 1..1341: mol_type = other DNA
gaggtgcagctgaaggagagcggccccggcctggtggcccccggcggcagcctgagcatcacctgcaccgtgagcggcttcagcctgaccgacagcagcatcaactgggtgcgccagccccccggcaagggcctggagtggctgggcatgatctggggcgacggccgcatcgactacgccgacgccctgaagagccgcctgagcatcagcaaggacagcagcaagagccaggtgttcctggagatgaccagcctgcgcaccgacgacaccgccacctactactgcgcccgcgacggctacttcccctacgccatggacttctggggccagggcaccagcgtgaccgtgagcagcgccagcaccaagggccccagcgtgttccccctggcccctagcagcaagagcacatctggcggcacagccgccctgggctgcctggtcaaggactacttccccgagcccgtgacagtgtcctggaactctggcgccctgaccagcggagtgcataccttccctgccgtgctgcagtccagcggcctgtacagcctgagcagcgtggtcacagtgcccagcagcagcctgggcacccagacctacatctgcaacgtgaaccacaagcccagcaacaccaaggtggacaagaaggtggaacccaagagctgcgacaagacccacacctgtcccccctgccctgcccctgaactgctgggcggaccctccgtgttcctgttccccccaaagcccaaggacaccctgatgatcagccggacccccgaagtgacctgcgtggtggtggacgtgtcccacgaggaccctgaagtgaagttcaattggtacgtggacggcgtggaagtgcataacgccaagaccaagcccagagaggaacagtacaacagcacctaccgggtggtgtccgtgctgaccgtgctgcaccaggactggctgaacggcaaagagtacaagtgcaaggtgtccaacaaggccctgcctgcccccatcgagaaaaccatcagcaaggccaagggccagcctagagagccccaagtctgcaccctgccccccagcagagatgagctgaccaagaaccaggtgtccctgagctgcgccgtgaagggcttctaccccagcgatatcgccgtggaatgggagagcaacggccagcccgagaacaactacaagaccaccccccctgtgctggacagcgacggctcattcttcctggtgtccaagctgacagtggacaagagccggtggcagcagggcaacgtgttcagctgcagcgtgatgcacgaggccctgcacaaccattacacccagaagtccctgagcctgagccccggc

SEQ ID NO: 78 - DNA, 651 bp, synthetic construct
  misc_feature 1..651: note = Synthetic Construct
  source 1..651: mol_type = other DNA
gacatcgtgctgacccagagccctgccagcctggccgtgtctctgggccagagagccaccatcagctgccgggccagcgagagcgtggacagctacggccagagctacatgcactggtatcagcagaaggccggccagccccccaagctgctgatctacctggccagcaacctggaaagcggcgtgcccgccagattcagcggcagcggcagcagaaccgacttcaccctgaccatcgaccccgtgcaggccgaggacgccgccacctactactgccagcagaacgccgaggacagccggaccttcggcggaggcaccaagctggaaatcaagggacagcccaaggctgccccctcggtcaccctgttccccccaagcagcgaggaactgcaggccaacaaggccaccctcgtgtgcctgatcagcgacttctaccctggcgccgtgaccgtggcctggaaggccgatagctctcccgtgaaggccggcgtggaaaccaccacccccagcaagcagagcaacaacaaatacgccgccagcagctacctgagcctgacccccgagcagtggaagtcccaccggtcctacagctgccaggtcacacacgagggcagcaccgtggaaaagaccgtggcccccaccgagtgcagc

SEQ ID NO: 79 - DNA, 1719 bp, synthetic construct
  misc_feature 1..1719: note = Synthetic Construct
  source 1..1719: mol_type = other DNA
caggtgcagctgcagcagagcggccctgagctggtcaagcctggcgccagcgtgaagatcagctgcaaggccagcggctacagcttcaccagctactggatccactggatcaagcagcggcctggccagggcctggaatggatcggcatgatcgaccccagcgacggcgagacacggctgaaccagagattccagggcagagccaccctgaccgtggacgagagcaccagcaccgcctacatgcagctgcggagccccaccagcgaggacagcgccgtgtactactgcacccggctgaaagagtacggcaactacgacagcttctacttcgacgtgtggggagccggcaccctggtcaccgtgtccagcgaagtgcagctggtggaaagcggcggaggcctggtgcagcccggcagaagcctgagactgagctgcgccgccagcggcttcaccttcgacgactacgccatgcactgggtccgacaggcccctggcaaaggactggaatgggtgtccgccatcacctggaacagcggccacatcgactacgccgacagcgtggaaggccggttcaccatcagccgggacaacgccaagaacagcctgtacctgcagatgaacagcctgcgggccgaggataccgccgtgtattattgcgccaaggtgtcctacctgagcaccgccagcagcctggactactggggccagggcaccctcgtgacagtgtcctccgcttccaccaagggccccagcgtgttccctctggcccctagcagcaagagcacatctggcggaacagccgccctgggctgcctggtcaaggactactttcccgagcccgtgaccgtgtcctggaactctggtgccctgacaagcggagtgcataccttccctgccgtgctgcagagcagcggcctgtactctctgagcagcgtggtcaccgtgccaagcagcagcctgggcacccagacctacatctgcaacgtgaaccacaagccctccaacaccaaggtggacaagaaggtggaacccaagagctgcgacaagacccacacctgtcctccctgtcctgcccctgaactgctgggcggaccctccgtgttcctgttccctccaaagcccaaggataccctgatgatcagccggacccctgaagtgacctgcgtggtggtggacgtgtcccacgaggatcccgaagtgaagttcaattggtacgtggacggcgtggaagtgcataacgccaagaccaagcccagagaggaacagtacaacagcacctaccgggtggtgtccgtgctgacagtgctgcaccaggactggctgaacggcaaagagtacaagtgcaaggtgtccaacaaggccctgccagcccctatcgagaaaaccatcagcaaggccaagggccagccccgcgagcctcaggtgtacacactgcctccatgccgggacgagctgaccaagaaccaggtgtccctgtggtgcctcgtgaagggcttctacccctccgatatcgccgtggaatgggagagcaacggccagcccgagaacaactacaagaccacccctcccgtgctggacagcgacggctcattcttcctgtacagcaagctgaccgtggacaagtcccggtggcagcagggcaacgtgttcagctgctctgtgatgcacgaggccctgcacaaccggttcacccagaagtccctgagcctgagccctggc

SEQ ID NO: 80 - DNA, 1023 bp, synthetic construct
  misc_feature 1..1023: note = Synthetic Construct
  source 1..1023: mol_type = other DNA
gacatccagatgacccagagccccagcagcctgagcgccagcgtgggcgacagagtgaccatcacctgtcgggccagccagggcatccggaactacctggcctggtatcagcagaagcccggcaaggcccccaagctgctgatctacgccgccagcacactgcagagcggcgtgcccagcagattcagcggcagcggctccggcaccgacttcaccctgaccatcagcagcctgcagcccgaggacgtggccacctactactgccagcggtacaacagagccccctacaccttcggccagggcaccaaggtggaaatcaagggcggctctggcagctccggcagcggcggagacattcagatgacacagtcccccgccagcctgtccgtgtccgtgggcgataccatcaccctgacatgccacgccagccagaacatcgacgtgtggctgagctggttccagcagaaacctggcaacatccctaagctgctcatctataaggccagcaacctgcacacaggcgtgccctccagattctccggctctggctctggcaccggctttacactgacaatcagttctctgcagcctgaggatatcgccacatattactgtcagcaggcccacagctaccctttcaccttcggaggcggcaccaagctcgagattaagggcggaagcggctcctccggctccggcggacgtacggtggccgctccttccgtgttcatcttccctccctccgacgagcagctgaagtccggcaccgcctccgtggtgtgtctgctgaacaacttctaccctcgggaggccaaggtgcagtggaaggtggacaacgccctgcagtccggcaactcccaggagtccgtcaccgagcaggactccaaggacagcacctactccctgtcctccaccctgaccctgtccaaggccgactacgagaagcacaaggtgtacgcctgtgaggtgacccaccagggcctgtccagccctgtgaccaagtccttcaaccggggcgagtgc

SEQ ID NO: 81 - protein, 573 aa, synthetic construct
  REGION 1..573: note = Synthetic Construct
EVQLVESGGGLVQPGRSLRLSCAASGFTFDDYAMHWVRQAPGKGLEWVSAITWNSGHIDYADSVEGRFTISRDNAKNSLYLQMNSLRAEDTAVYYCAKVSYLSTASSLDYWGQGTLVTVSSQVQLQQSGPELVKPGASVKISCKASGYSFTSYWIHWIKQRPGQGLEWIGMIDPSDGETRLNQRFQGRATLTVDESTSTAYMQLRSPTSEDSAVYYCTRLKEYGNYDSFYFDVWGAGTLVTVSSASTKGPSVFPLAPSSKSTSGGTAALGCLVKDYFPEPVTVSWNSGALTSGVHTFPAVLQSSGLYSLSSVVTVPSSSLGTQTYICNVNHKPSNTKVDKKVEPKSCDKTHTCPPCPAPELLGGPSVFLFPPKPKDTLMISRTPEVTCVVVDVSHEDPEVKFNWYVDGVEVHNAKTKPREEQYNSTYRVVSVLTVLHQDWLNGKEYKCKVSNKALPAPIEKTISKAKGQPREPQVYTLPPCRDELTKNQVSLWCLVKGFYPSDIAVEWESNGQPENNYKTTPPVLDSDGSFFLYSKLTVDKSRWQQGNVFSCSVMHEALHNRFTQKSLSLSPG

SEQ ID NO: 82 - protein, 341 aa, synthetic construct
  REGION 1..341: note = Synthetic Construct
DIQMTQSPASLSVSVGDTITLTCHASQNIDVWLSWFQQKPGNIPKLLIYKASNLHTGVPSRFSGSGSGTGFTLTISSLQPEDIATYYCQQAHSYPFTFGGGTKLEIKGGSGSSGSGGDIQMTQSPSSLSASVGDRVTITCRASQGIRNYLAWYQQKPGKAPKLLIYAASTLQSGVPSRFSGSGSGTDFTLTISSLQPEDVATYYCQRYNRAPYTFGQGTKVEIKGGSGSSGSGGRTVAAPSVFIFPPSDEQLKSGTASVVCLLNNFYPREAKVQWKVDNALQSGNSQESVTEQDSKDSTYSLSSTLTLSKADYEKHKVYACEVTHQGLSSPVTKSFNRGEC

SEQ ID NO: 83 - DNA, 1719 bp, synthetic construct
  misc_feature 1..1719: note = Synthetic Construct
  source 1..1719: mol_type = other DNA
gaggtgcagctggtggaaagcggcggaggactggtgcagcccggcagaagcctgagactgagctgcgccgccagcggcttcaccttcgacgactacgccatgcactgggtccgacaggcccctggcaagggcctggaatgggtgtccgccatcacctggaacagcggccacatcgactacgccgacagcgtggaaggccggttcaccatcagccgggacaacgccaagaacagcctgtacctgcagatgaacagcctgcgggccgaggacaccgccgtgtactactgcgccaaggtgtcctacctgagcaccgccagcagcctggactactggggccagggcaccctggtcaccgtgtccagtcaggtccagctgcagcagagcggccctgagctggtcaagcctggcgccagcgtgaagatcagctgcaaggccagcggctacagcttcaccagctactggatccactggatcaagcagcggcctggccagggcctcgagtggatcggcatgatcgaccccagcgacggcgagacacggctgaaccagagattccagggcagagccaccctgaccgtggacgagagcaccagcaccgcctacatgcagctgcggagccccaccagcgaggatagcgccgtgtattattgcacccggctgaaagagtacggcaactacgacagcttctacttcgacgtgtggggagccggcaccctcgtgacagtgtcctccgcttccaccaagggccccagcgtgttccctctggcccctagcagcaagagcacatctggcggaacagccgccctgggctgcctggtcaaggactactttcccgagcccgtgaccgtgtcctggaactctggtgccctgacaagcggagtgcataccttccctgccgtgctgcagagcagcggcctgtactctctgagcagcgtggtcaccgtgccaagcagcagcctgggcacccagacctacatctgcaacgtgaaccacaagccctccaacaccaaggtggacaagaaggtggaacccaagagctgcgacaagacccacacctgtcctccctgtcctgcccctgaactgctgggcggaccctccgtgttcctgttccctccaaagcccaaggataccctgatgatcagccggacccctgaagtgacctgcgtggtggtggacgtgtcccacgaggatcccgaagtgaagttcaattggtacgtggacggcgtggaagtgcataacgccaagaccaagcccagagaggaacagtacaacagcacctaccgggtggtgtccgtgctgacagtgctgcaccaggactggctgaacggcaaagagtacaagtgcaaggtgtccaacaaggccctgccagcccctatcgagaaaaccatcagcaaggccaagggccagccccgcgagcctcaggtgtacacactgcctccatgccgggacgagctgaccaagaaccaggtgtccctgtggtgcctcgtgaagggcttctacccctccgatatcgccgtggaatgggagagcaacggccagcccgagaacaactacaagaccacccctcccgtgctggacagcgacggctcattcttcctgtacagcaagctgaccgtggacaagtcccggtggcagcagggcaacgtgttcagctgctctgtgatgcacgaggccctgcacaaccggttcacccagaagtccctgagcctgagccctggc

SEQ ID NO: 84 - DNA, 1023 bp, synthetic construct
  misc_feature 1..1023: note = Synthetic Construct
  source 1..1023: mol_type = other DNA
gacatccagatgacccagagccccgccagcctgagcgtgtccgtgggcgataccatcaccctgacctgccacgccagccagaacatcgacgtgtggctgagctggttccagcagaagcccggcaacatccccaagctgctgatctacaaggccagcaacctgcacaccggcgtgcccagcagattcagcggctctggcagcggcaccggctttaccctgaccatcagcagcctgcagcccgaggatatcgccacctactactgccagcaggcccacagctaccccttcaccttcggcggaggcaccaagctggaaatcaagggcggcagcggcagctccggcagcggcggagacattcagatgacacagtcccccagcagcctgtccgccagcgtgggcgacagagtgaccatcacctgtcgggccagccagggcatccggaactacctggcctggtatcagcagaaacctggcaaggcccctaaactgctcatctacgccgccagcacactgcagtctggcgtgccctccagattctccggaagcggctccggcaccgatttcaccctgacaatctcatctctgcagcctgaggacgtggccacatattactgccagagatacaacagagccccctacacctttggccagggcaccaaggtcgagattaagggcggatccggctccagcggcagcggaggacgtacggtggccgctccttccgtgttcatcttccctccctccgacgagcagctgaagtccggcaccgcctccgtggtgtgtctgctgaacaacttctaccctcgggaggccaaggtgcagtggaaggtggacaacgccctgcagtccggcaactcccaggagtccgtcaccgagcaggactccaaggacagcacctactccctgtcctccaccctgaccctgtccaaggccgactacgagaagcacaaggtgtacgcctgtgaggtgacccaccagggcctgtccagccctgtgaccaagtccttcaaccggggcgagtgc

SEQ ID NO: 85 - protein, 452 aa, synthetic construct
  REGION 1..452: note = Synthetic Construct
QVQLQQSGPELVKPGASVKISCKASGYSFTSYWIHWIKQRPGQGLEWIGMIDPSDGETRLNQRFQGRATLTVDESTSTAYMQLRSPTSEDSAVYYCTRLKEYGNYDSFYFDVWGAGTLVTVSSASTKGPSVFPLAPSSKSTSGGTAALGCLVKDYFPEPVTVSWNSGALTSGVHTFPAVLQSSGLYSLSSVVTVPSSSLGTQTYICNVNHKPSNTKVDKKVEPKSCDKTHTCPPCPAPELLGGPSVFLFPPKPKDTLMISRTPEVTCVVVDVSHEDPEVKFNWYVDGVEVHNAKTKPREEQYNSTYRVVSVLTVLHQDWLNGKEYKCKVSNKALPAPIEKTISKAKGQPREPQVCTLPPSRDELTKNQVSLSCAVKGFYPSDIAVEWESNGQPENNYKTTPPVLDSDGSFFLVSKLTVDKSRWQQGNVFSCSVMHEALHNHYTQKSLSLSPG

SEQ ID NO: 86 - protein, 213 aa, synthetic construct
  REGION 1..213: note = Synthetic Construct
DIQMTQSPASLSVSVGDTITLTCHASQNIDVWLSWFQQKPGNIPKLLIYKASNLHTGVPSRFSGSGSGTGFTLTISSLQPEDIATYYCQQAHSYPFTFGGGTKLEIKGQPKAAPSVTLFPPSSEELQANKATLVCLISDFYPGAVTVAWKADSSPVKAGVETTTPSKQSNNKYAASSYLSLTPEQWKSHRSYSCQVTHEGSTVEKTVAPTECS

SEQ ID NO: 87 - protein, 568 aa, synthetic construct
  REGION 1..568: note = Synthetic Construct
EVQLKESGPGLVAPGGSLSITCTVSGFSLTDSSINWVRQPPGKGLEWLGMIWGDGRIDYADALKSRLSISKDSSKSQVFLEMTSLRTDDTATYYCARDGYFPYAMDFWGQGTSVTVSSEVQLVESGGGLVQPGRSLRLSCAASGFTFDDYAMHWVRQAPGKGLEWVSAITWNSGHIDYADSVEGRFTISRDNAKNSLYLQMNSLRAEDTAVYYCAKVSYLSTASSLDYWGQGTLVTVSSASTKGPSVFPLAPSSKSTSGGTAALGCLVKDYFPEPVTVSWNSGALTSGVHTFPAVLQSSGLYSLSSVVTVPSSSLGTQTYICNVNHKPSNTKVDKKVEPKSCDKTHTCPPCPAPELLGGPSVFLFPPKPKDTLMISRTPEVTCVVVDVSHEDPEVKFNWYVDGVEVHNAKTKPREEQYNSTYRVVSVLTVLHQDWLNGKEYKCKVSNKALPAPIEKTISKAKGQPREPQVYTLPPCRDELTKNQVSLWCLVKGFYPSDIAVEWESNGQPENNYKTTPPVLDSDGSFFLYSKLTVDKSRWQQGNVFSCSVMHEALHNRFTQKSLSLSPG

SEQ ID NO: 88 - protein, 344 aa, synthetic construct
  REGION 1..344: note = Synthetic Construct
IQMTQSPSSLSASVGDRVTITCRASQGIRNYLAWYQQKPGKAPKLLIYAASTLQSGVPSRFSGSGSGTDFTLTISSLQPEDVATYYCQRYNRAPYTFGQGTKVEIKGGSGSSGSGGDIVLTQSPASLAVSLGQRATISCRASESVDSYGQSYMHWYQQKAGQPPKLLIYLASNLESGVPARFSGSGSRTDFTLTIDPVQAEDAATYYCQQNAEDSRTFGGGTKLEIKGGSGSSGSGGRTVAAPSVFIFPPSDEQLKSGTASVVCLLNNFYPREAKVQWKVDNALQSGNSQESVTEQDSKDSTYSLSSTLTLSKADYEKHKVYACEVTHQGLSSPVTKSFNRGEC

SEQ ID NO: 89 - DNA, 1356 bp, synthetic construct
  misc_feature 1..1356: note = Synthetic Construct
  source 1..1356: mol_type = other DNA
caggtgcagctgcagcagagcggccccgagctggtgaagcccggcgccagcgtgaagatcagctgcaaggccagcggctacagcttcaccagctactggattcactggatcaagcagcgccccggccagggcctggagtggatcggcatgatcgaccccagcgacggcgagacccgcctgaaccagcgcttccagggccgcgccaccctgaccgtggacgagagcaccagcaccgcctacatgcagctgcgcagccccaccagcgaggacagcgccgtgtactactgcacccgcctgaaggagtacggcaactacgacagcttctacttcgacgtgtggggcgccggcaccctggtgaccgtgagcagcgccagcaccaagggccccagcgtgttccccctggcccctagcagcaagagcacatctggcggcacagccgccctgggctgcctggtcaaggactacttccccgagcccgtgacagtgtcctggaactctggcgccctgaccagcggagtgcataccttccctgccgtgctgcagtccagcggcctgtacagcctgagcagcgtggtcacagtgcccagcagcagcctgggcacccagacctacatctgcaacgtgaaccacaagcccagcaacaccaaggtggacaagaaggtggaacccaagagctgcgacaagacccacacctgtcccccctgccctgcccctgaactgctgggcggaccctccgtgttcctgttccccccaaagcccaaggacaccctgatgatcagccggacccccgaagtgacctgcgtggtggtggacgtgtcccacgaggaccctgaagtgaagttcaattggtacgtggacggcgtggaagtgcataacgccaagaccaagcccagagaggaacagtacaacagcacctaccgggtggtgtccgtgctgaccgtgctgcaccaggactggctgaacggcaaagagtacaagtgcaaggtgtccaacaaggccctgcctgcccccatcgagaaaaccatcagcaaggccaagggccagcctagagagccccaagtctgcaccctgccccccagcagagatgagctgaccaagaaccaggtgtccctgagctgcgccgtgaagggcttctaccccagcgatatcgccgtggaatgggagagcaacggccagcccgagaacaactacaagaccaccccccctgtgctggacagcgacggctcattcttcctggtgtccaagctgacagtggacaagagccggtggcagcagggcaacgtgttcagctgcagcgtgatgcacgaggccctgcacaaccattacacccagaagtccctgagcctgagccccggc

SEQ ID NO: 90 - DNA, 639 bp, synthetic construct
  misc_feature 1..639: note = Synthetic Construct
  source 1..639: mol_type = other DNA
gacatccagatgacccagagccccgccagcctgagcgtgtccgtgggcgataccatcaccctgacctgccacgccagccagaacatcgacgtgtggctgagctggttccagcagaagcccggcaacatccccaagctgctgatctacaaggccagcaacctgcacaccggcgtgcccagcagattcagcggctctggcagcggcaccggctttaccctgaccatcagcagcctgcagcccgaggatatcgccacctactactgccagcaggcccacagctaccccttcaccttcggcggaggcaccaagctggaaatcaagggacagcccaaggctgccccctcggtcaccctgttccccccaagctctgaggaactgcaggccaacaaggccaccctcgtgtgcctgatcagcgacttctaccctggcgccgtgaccgtggcctggaaggccgatagctctcccgtgaaggccggcgtggaaaccaccacccccagcaagcagagcaacaacaaatacgccgccagcagctacctgagcctgacccccgagcagtggaagtcccaccggtcctacagctgccaggtcacacacgagggcagcaccgtggaaaagaccgtggcccccaccgagtgcagc

SEQ ID NO: 91 - DNA, 1704 bp, synthetic construct
  misc_feature 1..1704: note = Synthetic Construct
  source 1..1704: mol_type = other DNA
gaggtgcagctgaaagagtccggccctggactggtggcccctggcggcagcctgagcatcacctgtaccgtgtccggcttcagcctgaccgacagcagcatcaactgggtccgacagccccctggcaagggcctggaatggctgggcatgatctggggcgacggccggatcgactacgccgacgccctgaagtcccggctgagcatcagcaaggacagcagcaagagccaggtgttcctggaaatgaccagcctgcggaccgacgacaccgccacctactactgcgccagggacggctacttcccctacgccatggatttctggggccagggcaccagcgtgaccgtgtcctccgaagtgcagctggtggaaagcggcggaggcctggtgcagcccggcagaagcctgagactgagctgcgccgccagcggcttcaccttcgacgactacgccatgcactgggtccgccaggctcccggaaagggactcgagtgggtgtccgccatcacctggaacagcggccacatcgattacgccgatagcgtggaaggccggttcaccatcagccgggacaacgccaagaacagcctgtacctgcagatgaacagcctgagagccgaggataccgccgtgtactactgtgccaaggtgtcctacctgagcaccgccagcagcctggactactggggacagggaaccctggtcaccgtgtccagcgcttccaccaagggccccagcgtgttccctctggcccctagcagcaagagcacatctggcggaacagccgccctgggctgcctggtcaaggactactttcccgagcccgtgaccgtgtcctggaactctggtgccctgacaagcggagtgcataccttccctgccgtgctgcagagcagcggcctgtactctctgagcagcgtggtcaccgtgccaagcagcagcctgggcacccagacctacatctgcaacgtgaaccacaagccctccaacaccaaggtggacaagaaggtggaacccaagagctgcgacaagacccacacctgtcctccctgtcctgcccctgaactgctgggcggaccctccgtgttcctgttccctccaaagcccaaggataccctgatgatcagccggacccctgaagtgacctgcgtggtggtggacgtgtcccacgaggatcccgaagtgaagttcaattggtacgtggacggcgtggaagtgcataacgccaagaccaagcccagagaggaacagtacaacagcacctaccgggtggtgtccgtgctgacagtgctgcaccaggactggctgaacggcaaagagtacaagtgcaaggtgtccaacaaggccctgccagcccctatcgagaaaaccatcagcaaggccaagggccagccccgcgagcctcaggtgtacacactgcctccatgccgggacgagctgaccaagaaccaggtgtccctgtggtgcctcgtgaagggcttctacccctccgatatcgccgtggaatgggagagcaacggccagcccgagaacaactacaagaccacccctcccgtgctggacagcgacggctcattcttcctgtacagcaagctgaccgtggacaagtcccggtggcagcagggcaacgtgttcagctgctctgtgatgcacgaggccctgcacaaccggttcacccagaagtccctgagcctgagccctggc

SEQ ID NO: 92 - DNA, 1035 bp, synthetic construct
  misc_feature 1..1035: note = Synthetic Construct
  source 1..1035: mol_type = other DNA
gacatccagatgacccagagccccagcagcctgagcgccagcgtgggcgacagagtgaccatcacctgtcgggccagccagggcatccggaactacctggcctggtatcagcagaagcccggcaaggcccccaagctgctgatctacgccgccagcacactgcagagcggcgtgcccagcagattcagcggcagcggctccggcaccgacttcaccctgaccatcagcagcctgcagcccgaggacgtggccacctactactgccagcggtacaacagagccccctacaccttcggccagggcaccaaggtggaaatcaagggcggctctggcagctccggctctggcggcgatatcgtgctgacccagtctcccgccagcctggccgtgtctctgggccagagagccaccatcagctgcagagccagcgagagcgtggacagctacggccagagctacatgcattggtatcagcagaaagccggccagcctcctaaactgctcatctacctggccagcaacctggaatccggcgtgcccgccaggttttccggcagcggcagcagaaccgatttcacactgacaatcgaccccgtgcaggccgaggatgccgccacatattactgtcagcagaacgccgaggacagccggaccttcggcggaggcaccaagctcgagattaagggcggaagcggctccagcggcagtggcggacgtacggtggccgctccttccgtgttcatcttccctccctccgacgagcagctgaagtccggcaccgcctccgtggtgtgtctgctgaacaacttctaccctcgggaggccaaggtgcagtggaaggtggacaacgccctgcagtccggcaactcccaggagtccgtcaccgagcaggactccaaggacagcacctactccctgtcctccaccctgaccctgtccaaggccgactacgagaagcacaaggtgtacgcctgtgaggtgacccaccagggcctgtccagccctgtgaccaagtccttcaaccggggcgagtgc

SEQ ID NO: 93 - protein, 568 aa, synthetic construct
  REGION 1..568: note = Synthetic Construct
EVQLVESGGGLVQPGRSLRLSCAASGFTFDDYAMHWVRQAPGKGLEWVSAITWNSGHIDYADSVEGRFTISRDNAKNSLYLQMNSLRAEDTAVYYCAKVSYLSTASSLDYWGQGTLVTVSSEVQLKESGPGLVAPGGSLSITCTVSGFSLTDSSINWVRQPPGKGLEWLGMIWGDGRIDYADALKSRLSISKDSSKSQVFLEMTSLRTDDTATYYCARDGYFPYAMDFWGQGTSVTVSSASTKGPSVFPLAPSSKSTSGGTAALGCLVKDYFPEPVTVSWNSGALTSGVHTFPAVLQSSGLYSLSSVVTVPSSSLGTQTYICNVNHKPSNTKVDKKVEPKSCDKTHTCPPCPAPELLGGPSVFLFPPKPKDTLMISRTPEVTCVVVDVSHEDPEVKFNWYVDGVEVHNAKTKPREEQYNSTYRVVSVLTVLHQDWLNGKEYKCKVSNKALPAPIEKTISKAKGQPREPQVYTLPPCRDELTKNQVSLWCLVKGFYPSDIAVEWESNGQPENNYKTTPPVLDSDGSFFLYSKLTVDKSRWQQGNVFSCSVMHEALHNRFTQKSLSLSPG

SEQ ID NO: 94 - protein, 345 aa, synthetic construct
  REGION 1..345: note = Synthetic Construct
DIVLTQSPASLAVSLGQRATISCRASESVDSYGQSYMHWYQQKAGQPPKLLIYLASNLESGVPARFSGSGSRTDFTLTIDPVQAEDAATYYCQQNAEDSRTFGGGTKLEIKGGSGSSGSGGDIQMTQSPSSLSASVGDRVTITCRASQGIRNYLAWYQQKPGKAPKLLIYAASTLQSGVPSRFSGSGSGTDFTLTISSLQPEDVATYYCQRYNRAPYTFGQGTKVEIKGGSGSSGSGGRTVAAPSVFIFPPSDEQLKSGTASVVCLLNNFYPREAKVQWKVDNALQSGNSQESVTEQDSKDSTYSLSSTLTLSKADYEKHKVYACEVTHQGLSSPVTKSFNRGEC

SEQ ID NO: 95 - DNA, 1704 bp, synthetic construct
  misc_feature 1..1704: note = Synthetic Construct
  source 1..1704: mol_type = other DNA
gaggtgcagctggtggaaagcggcggaggactggtgcagcccggcagaagcctgagactgagctgcgccgccagcggcttcaccttcgacgactacgccatgcactgggtccgacaggcccctggcaagggcctggaatgggtgtccgccatcacctggaacagcggccacatcgactacgccgacagcgtggaaggccggttcaccatcagccgggacaacgccaagaacagcctgtacctgcagatgaacagcctgcgggccgaggacaccgccgtgtactactgcgccaaggtgtcctacctgagcaccgccagcagcctggactactggggccagggcaccctggtcaccgtgtcctccgaagtgcagctgaaagagtccggccctggcctggtggcccctggcggcagcctgagcatcacctgtaccgtgtccggcttcagcctgaccgacagcagcatcaactgggtccgccagcctcccggaaagggactcgagtggctgggcatgatctggggcgacggccggatcgattacgccgatgccctgaagtcccggctgagcatcagcaaggacagcagcaagagccaggtgttcctggaaatgaccagcctgagaaccgacgacaccgccacctactactgtgcccgggacggctacttcccctacgccatggatttctggggacagggaaccagcgtgaccgtgtccagcgcttccaccaagggccccagcgtgttccctctggcccctagcagcaagagcacatctggcggaacagccgccctgggctgcctggtcaaggactactttcccgagcccgtgaccgtgtcctggaactctggtgccctgacaagcggagtgcataccttccctgccgtgctgcagagcagcggcctgtactctctgagcagcgtggtcaccgtgccaagcagcagcctgggcacccagacctacatctgcaacgtgaaccacaagccctccaacaccaaggtggacaagaaggtggaacccaagagctgcgacaagacccacacctgtcctccctgtcctgcccctgaactgctgggcggaccctccgtgttcctgttccctccaaagcccaaggataccctgatgatcagccggacccctgaagtgacctgcgtggtggtggacgtgtcccacgaggatcccgaagtgaagttcaattggtacgtggacggcgtggaagtgcataacgccaagaccaagcccagagaggaacagtacaacagcacctaccgggtggtgtccgtgctgacagtgctgcaccaggactggctgaacggcaaagagtacaagtgcaaggtgtccaacaaggccctgccagcccctatcgagaaaaccatcagcaaggccaagggccagccccgcgagcctcaggtgtacacactgcctccatgccgggacgagctgaccaagaaccaggtgtccctgtggtgcctcgtgaagggcttctacccctccgatatcgccgtggaatgggagagcaacggccagcccgagaacaactacaagaccacccctcccgtgctggacagcgacggctcattcttcctgtacagcaagctgaccgtggacaagtcccggtggcagcagggcaacgtgttcagctgctctgtgatgcacgaggccctgcacaaccggttcacccagaagtccctgagcctgagccctggc

SEQ ID NO: 96 - DNA, 1035 bp, synthetic construct
  misc_feature 1..1035: note = Synthetic Construct
  source 1..1035: mol_type = other DNA
gacatcgtgctgacccagagccctgccagcctggccgtgtctctgggccagagagccaccatcagctgccgggccagcgagagcgtggacagctacggccagagctacatgcactggtatcagcagaaggccggccagccccccaagctgctgatctacctggccagcaacctggaaagcggcgtgcccgccagattcagcggcagcggcagcagaaccgacttcaccctgaccatcgaccccgtgcaggccgaggacgccgccacctactactgccagcagaacgccgaggacagccggaccttcggcggaggcaccaagctggaaatcaagggcggctccggcagcagcggctctggcggcgatatccagatgacccagtcccccagcagcctgagcgccagcgtgggcgacagagtgaccatcacctgtagagccagccagggcatccggaactacctggcttggtatcagcagaaacccggaaaggcccctaaactgctcatctacgccgccagcaccctgcagtccggcgtgccaagcagattctccggctctggcagcggcaccgatttcacactgacaatcagcagcctgcagcccgaggatgtggccacctattattgccagagatacaacagagccccctacaccttcggccagggcaccaaggtcgagattaagggcggaagcggcagctccggctccggcggacgtacggtggccgctccttccgtgttcatcttccctccctccgacgagcagctgaagtccggcaccgcctccgtggtgtgtctgctgaacaacttctaccctcgggaggccaaggtgcagtggaaggtggacaacgccctgcagtccggcaactcccaggagtccgtcaccgagcaggactccaaggacagcacctactccctgtcctccaccctgaccctgtccaaggccgactacgagaagcacaaggtgtacgcctgtgaggtgacccaccagggcctgtccagccctgtgaccaagtccttcaaccggggcgagtgc

SEQ ID NO: 97 - DNA, 1710 bp, synthetic construct
  misc_feature 1..1710: note = Synthetic Construct
  source 1..1710: mol_type = other DNA
gaggtgcagctgaaagagtccggccctggactggtggcccctggcggcagcctgagcatcacctgtaccgtgtccggcttcagcctgaccgacagcagcatcaactgggtccgacagccccctggcaagggcctggaatggctgggcatgatctggggcgacggccggatcgactacgccgacgccctgaagtcccggctgagcatcagcaaggacagcagcaagagccaggtgttcctggaaatgaccagcctgcggaccgacgacaccgccacctactactgcgccagggacggctacttcccctacgccatggatttctggggccagggcaccagcgtgaccgtgtccagtcaggtccagctgcagcagagcggccctgagctggtcaagcctggcgccagcgtgaagatcagctgcaaggccagcggctacagcttcaccagctactggatccactggatcaagcagcggcctggccagggcctcgagtggatcggaatgatcgaccccagcgacggcgagacacggctgaaccagagattccagggcagagccaccctgaccgtggacgagagcaccagcaccgcctacatgcagctgcggagccccaccagcgaggacagcgccgtgtactactgcacccggctgaaagaatacggcaactacgacagcttctacttcgacgtgtggggagccggcaccctggtcaccgtgtctagcgcttccaccaagggccccagcgtgttccctctggcccctagcagcaagagcacatctggcggaacagccgccctgggctgcctggtcaaggactactttcccgagcccgtgaccgtgtcctggaactctggtgccctgacaagcggagtgcataccttccctgccgtgctgcagagcagcggcctgtactctctgagcagcgtggtcaccgtgccaagcagcagcctgggcacccagacctacatctgcaacgtgaaccacaagccctccaacaccaaggtggacaagaaggtggaacccaagagctgcgacaagacccacacctgtcctccctgtcctgcccctgaactgctgggcggaccctccgtgttcctgttccctccaaagcccaaggataccctgatgatcagccggacccctgaagtgacctgcgtggtggtggacgtgtcccacgaggatcccgaagtgaagttcaattggtacgtggacggcgtggaagtgcataacgccaagaccaagcccagagaggaacagtacaacagcacctaccgggtggtgtccgtgctgacagtgctgcaccaggactggctgaacggcaaagagtacaagtgcaaggtgtccaacaaggccctgccagcccctatcgagaaaaccatcagcaaggccaagggccagccccgcgagcctcaggtgtacacactgcctccatgccgggacgagctgaccaagaaccaggtgtccctgtggtgcctcgtgaagggcttctacccctccgatatcgccgtggaatgggagagcaacggccagcccgagaacaactacaagaccacccctcccgtgctggacagcgacggctcattcttcctgtacagcaagctgaccgtggacaagtcccggtggcagcagggcaacgtgttcagctgctctgtgatgcacgaggccctgcacaaccggttcacccagaagtccctgagcctgagccctggc

SEQ ID NO: 98 - protein, 4 aa, synthetic construct
  REGION 1..4: note = Synthetic Construct
GGGG

SEQ ID NO: 99 - protein, 5 aa, synthetic construct
  REGION 1..5: note = Synthetic Construct
GGGGG

SEQ ID NO: 100 - protein, 6 aa, synthetic construct
  REGION 1..6: note = Synthetic Construct
GGGGGG

SEQ ID NO: 101 - protein, 7 aa, synthetic construct
  REGION 1..7: note = Synthetic Construct
GGGGGGG

SEQ ID NO: 102 - protein, 8 aa, synthetic construct
  REGION 1..8: note = Synthetic Construct
GGGGGGGG

SEQ ID NO: 103 - protein, 5 aa, synthetic construct
  REGION 1..5: note = Synthetic Construct
GGGGS

SEQ ID NO: 104 - protein, 10 aa, synthetic construct
  REGION 1..10: note = Synthetic Construct
GGGGSGGGGS

SEQ ID NO: 105 - protein, 15 aa, synthetic construct
  REGION 1..15: note = Synthetic Construct
GGGGSGGGGSGGGGS

SEQ ID NO: 106 - protein, 5 aa, synthetic construct
  REGION 1..5: note = Synthetic Construct
TKGPS

SEQ ID NO: 107 - protein, 5 aa, synthetic construct
  REGION 1..5: note = Synthetic Construct
TVAAP

SEQ ID NO: 108 - protein, 5 aa, synthetic construct
  REGION 1..5: note = Synthetic Construct
QPKAA

SEQ ID NO: 109 - protein, 5 aa, synthetic construct
  REGION 1..5: note = Synthetic Construct
QRIEG

SEQ ID NO: 110 - protein, 7 aa, synthetic construct
  REGION 1..7: note = Synthetic Construct
ASTKGPS

SEQ ID NO: 111 - protein, 7 aa, synthetic construct
  REGION 1..7: note = Synthetic Construct
RTVAAPS

SEQ ID NO: 112 - protein, 7 aa, synthetic construct
  REGION 1..7: note = Synthetic Construct
GQPKAAP

SEQ ID NO: 113 - protein, 7 aa, synthetic construct
  REGION 1..7: note = Synthetic Construct
HIDSPNK

SEQ ID NO: 114 - protein, 448 aa, synthetic construct
  REGION 1..448: note = Synthetic Construct
QVQLQQPGAELVKPGASVKMSCKASGYTFTSYNMHWVKQTPGRGLEWIGAIYPGNGDTSYNQKFKGKATLTADKSSSTAYMQLSSLTSEDSAVYYCARSTYYGGDWYFNVWGAGTTVTVSAASTKGPSVFPLAPCSRSTSESTAALGCLVKDYFPEPVTVSWNSGALTSGVHTFPAVLQSSGLYSLSSVVTVPSSSLGTKTYTCNVDHKPSNTKVDKRVESKYGPPCPPCPAPEFLGGPSVFLFPPKPKDTLMISRTPEVTCVVVDVSQEDPEVQFNWYVDGVEVHNAKTKPREEQFNSTYRVVSVLTVLHQDWLNGKEYKCKVSNKGLPSSIEKTISKAKGQPREPQVYTLPPCQEEMTKNQVSLWCLVKGFYPSDIAVEWESNGQPENNYKTTPPVLDSDGSFFLYSKLTVDKSRWQEGNVFSCSVMHEALHNHYTQKSLSLSLGK

SEQ ID NO: 115 - protein, 213 aa, synthetic construct
  REGION 1..213: note = Synthetic Construct
QIVLSQSPAILSASPGEKVTMTCRASSSVSYIHWFQQKPGSSPKPWIYATSNLASGVPVRFSGSGSGTSYSLTISRVEAEDAATYYCQQWTSNPPTFGGGTKLEIKRTVAAPSVFIFPPSDEQLKSGTASVVCLLNNFYPREAKVQWKVDNALQSGNSQESVTEQDSKDSTYSLSSTLTLSKADYEKHKVYACEVTHQGLSSPVTKSFNRGEC

SEQ ID NO: 116 - DNA, 1344 bp, synthetic construct
  misc_feature 1..1344: note = Synthetic Construct
  source 1..1344: mol_type = other DNA
caggtgcagctgcagcagcctggcgccgaactcgtgaaacctggcgcctccgtgaagatgagctgcaaggccagcggctacaccttcaccagctacaacatgcactgggtcaagcagacccccggcagaggcctggaatggatcggcgccatctaccccggcaacggcgacacctcctacaaccagaagttcaagggcaaggccaccctgaccgccgacaagagcagcagcacagcctacatgcagctgtccagcctgaccagcgaggacagcgccgtgtactactgcgccagaagcacctactacggcggcgactggtacttcaacgtgtggggagccggcaccaccgtgacagtgtctgctgcttcgaccaagggcccatcggtgttccctctggccccttgcagcagaagcaccagcgaatctacagccgccctgggctgcctcgtgaaggactactttcccgagcccgtgaccgtgtcctggaactctggcgctctgacaagcggcgtgcacacctttccagccgtgctccagagcagcggcctgtactctctgagcagcgtcgtgacagtgcccagcagcagcctgggcaccaagacctacacctgtaacgtggaccacaagcccagcaacaccaaggtggacaagcgggtggaatctaagtacggccctccctgccctccttgcccagcccctgaatttctgggcggaccctccgtgttcctgttccccccaaagcccaaggacaccctgatgatcagccggacccccgaagtgacctgcgtggtggtggatgtgtcccaggaagatcccgaggtgcagttcaattggtacgtggacggcgtggaagtgcacaacgccaagaccaagcccagagaggaacagttcaacagcacctaccgggtggtgtccgtgctgaccgtgctgcaccaggactggctgaacggcaaagagtacaagtgcaaggtgtccaacaagggcctgcccagctccatcgagaaaaccatcagcaaggccaagggccagccccgcgagcctcaagtgtataccctgcccccttgccaggaagagatgaccaagaaccaggtgtccctgtggtgtctcgtgaaaggcttctaccccagcgacattgccgtggaatgggagagcaacggccagcccgagaacaactacaagaccaccccccctgtgctggacagcgacggctcattcttcctgtactccaagctgaccgtggacaagagccggtggcaggaaggcaacgtgttcagctgctccgtgatgcacgaggccctgcacaaccactacacccagaagtccctgtctctgtccctgggcaag

SEQ ID NO: 117 - DNA, 639 bp, synthetic construct
  misc_feature 1..639: note = Synthetic Construct
  source 1..639: mol_type = other DNA
cagatcgtgctgagccagagccctgccatcctgagcgcttccccaggcgagaaagtgaccatgacctgcagagccagcagcagcgtgtcctacatccactggttccagcagaagcccggcagcagccccaagccttggatctacgccaccagcaatctggccagcggagtgcctgtgcggtttagcggctctggcagcggcacaagctacagcctgaccatcagccgggtggaagccgaagatgccgccacctactactgccagcagtggaccagcaacccccccacatttggcggaggcaccaagctggaaatcaagcgtacggtggccgctcccagcgtgttcatcttcccacctagcgacgagcagctgaagtccggcacagcctctgtcgtgtgcctgctgaacaacttctacccccgcgaggccaaagtgcagtggaaggtggacaacgccctgcagagcggcaacagccaggaaagcgtgaccgagcaggacagcaaggactccacctacagcctgagcagcaccctgacactgagcaaggccgactacgagaagcacaaggtgtacgcctgcgaagtgacccaccagggcctgtctagccccgtgaccaagagcttcaaccggggcgagtgt

SEQ ID NO: 118 - DNA, 1713 bp, synthetic construct; identical to SEQ ID NO: 11
  misc_feature 1..1713: note = Synthetic Construct
  source 1..1713: mol_type = other DNA

SEQ ID NO: 119 - DNA, 1026 bp, synthetic construct; identical to SEQ ID NO: 12
  misc_feature 1..1026: note = Synthetic Construct
  source 1..1026: mol_type = other DNA

SEQ ID NO: 120 - protein, 8 aa, synthetic construct
  REGION 1..8: note = Synthetic Construct
GYTFTSYN

SEQ ID NO: 121 - protein, 8 aa, synthetic construct
  REGION 1..8: note = Synthetic Construct
IYPGNGDT

SEQ ID NO: 122 - protein, 14 aa, synthetic construct
  REGION 1..14: note = Synthetic Construct
ARSTYYGGDWYFNV

SEQ ID NO: 123 - protein, 5 aa, synthetic construct
  REGION 1..5: note = Synthetic Construct
SSVSY

SEQ ID NO: 124 - skipped

SEQ ID NO: 125 - protein, 7 aa, synthetic construct
  REGION 1..7: note = Synthetic Construct
QQWTSNP

SEQ ID NO: 126 - protein, 10 aa, synthetic construct
  REGION 1..10: note = Synthetic Construct
GYIFTNYNIH

SEQ ID NO: 127 - protein, 10 aa, synthetic construct
  REGION 1..10: note = Synthetic Construct
AIYPGNGDAP

SEQ ID NO: 128 - protein, 9 aa, synthetic construct
  REGION 1..9: note = Synthetic Construct
ANWDVAFAY

SEQ ID NO: 129 - protein, 10 aa, synthetic construct
  REGION 1..10: note = Synthetic Construct
GFTFDDYAMH

SEQ ID NO: 130 - protein, 10 aa, synthetic construct
  REGION 1..10: note = Synthetic Construct
AITWNSGHID

SEQ ID NO: 131 - protein, 12 aa, synthetic construct
  REGION 1..12: note = Synthetic Construct
VSYLSTASSLDY

SEQ ID NO: 132 - protein, 10 aa, synthetic construct
  REGION 1..10: note = Synthetic Construct
GYSFTSYWIH

SEQ ID NO: 133 - protein, 9 aa, synthetic construct
  REGION 1..9: note = Synthetic Construct
MIDPSDGET

SEQ ID NO: 134 - protein, 14 aa, synthetic construct
  REGION 1..14: note = Synthetic Construct
LKEYGNYDSFYFDV

SEQ ID NO: 135 - protein, 10 aa, synthetic construct
  REGION 1..10: note = Synthetic Construct
GFSLTDSSIN

SEQ ID NO: 136 - protein, 9 aa, synthetic construct
  REGION 1..9: note = Synthetic Construct
MIWGDGRID

SEQ ID NO: 137 - protein, 10 aa, synthetic construct
  REGION 1..10: note = Synthetic Construct
DGYFPYAMDF

SEQ ID NO: 138 - protein, 11 aa, synthetic construct
  REGION 1..11: note = Synthetic Construct
KASQDIDRYMA

SEQ ID NO: 139 - protein, 7 aa, synthetic construct
  REGION 1..7: note = Synthetic Construct
DTSTLQS

SEQ ID NO: 140 - protein, 8 aa, synthetic construct
  REGION 1..8: note = Synthetic Construct
LQYDNLWT

SEQ ID NO: 141 - protein, 11 aa, synthetic construct
  REGION 1..11: note = Synthetic Construct
RASQGIRNYLA

SEQ ID NO: 142 - protein, 9 aa, synthetic construct
  REGION 1..9: note = Synthetic Construct
QRYNRAPYT

SEQ ID NO: 143 - protein, 11 aa, synthetic construct
  REGION 1..11: note = Synthetic Construct
HASQNIDVWLS

SEQ ID NO: 144 - protein, 9 aa, synthetic construct
  REGION 1..9: note = Synthetic Construct
QQAHSYPFT

SEQ ID NO: 145 - protein, 15 aa, synthetic construct
  REGION 1..15: note = Synthetic Construct
RASESVDSYGQSYMH

SEQ ID NO: 146 - protein, 7 aa, synthetic construct
  REGION 1..7: note = Synthetic Construct
LASNLES

SEQ ID NO: 147 - protein, 9 aa, synthetic construct
  REGION 1..9: note = Synthetic Construct
QQNAEDSRT

SEQ ID NO: 148 - protein, 10 aa, synthetic construct
  REGION 1..10: note = Synthetic Construct
GGSGSSGSGG

SEQ ID NO: 149 - protein, 11 aa, synthetic construct
  REGION 1..11: note = Synthetic Construct
QSLVHNNGNTY

SEQ ID NO: 150 - protein, 120 aa, synthetic construct [sequence omitted]

SEQ ID NO: 151 - protein, 107 aa, synthetic construct [sequence omitted]

SEQ ID NO: 152 - protein, 121 aa, synthetic construct
  REGION 1..121: note = Synthetic Construct
QVQLVESGGGVVQPGRSLRLSCAASGFTFTKAWMHWVRQAPGKQLEWVAQIKDKSNSYATYYADSVKGRFTISRDDSKNTLYLQMNSLRAEDTAVYYCRGVYYALSPFDYWGQGTLVTVSS

SEQ ID NO: 153 - protein, 112 aa, synthetic construct
  REGION 1..112: note = Synthetic Construct
DIVMTQTPLSLSVTPGQPASISCKSSQSLVHNNANTYLSWYLQKPGQSPQSLIYKVSNRFSGVPDRFSGSGSGTDFTLKISRVEAEDVGVYYCGQGTQYPFTFGSGTKVEIK

SEQ ID NO: 154 - protein, 121 aa, synthetic construct
  REGION 1..121: note = Synthetic Construct
QVQLVESGGGVVQPGRSLRLSCAASGFTFTKAWMHWVRQAPGKGLEWVAQIKDKSNSYATYYADSVKGRFTISRDNSKNTLYLQMNSLRAEDTAVYYCRGVYYALSPFDYWGQGTLVTVSS

SEQ ID NO: 155 - protein, 112 aa, synthetic construct
  REGION 1..112: note = Synthetic Construct
DIVMTQTPLSLSVTPGQPASISCKSSQSLVHNNGNTYLSWYLQKPGQSPQLLIYKVSNRFSGVPDRFSGSGSGTDFTLKISRVEAEDVGVYYCGQGTQYPFTFGGGTKVEIK

SEQ ID NO: 156 - protein, 124 aa, synthetic construct
  REGION 1..124: note = Synthetic Construct
QVQLVQSGAEVKKPGSSVKVSCKASGYAFSSYWMNWVRQAPGQGLEWIGQIWPGDGDTNYNQKFKGRATLTADESTSTAYMELSSLRSEDTAVYYCARRETTTVGRYYYAMDYWGQGTTVTVSS

SEQ ID NO: 157 - protein, 111 aa, synthetic construct
  REGION 1..111: note = Synthetic Construct
DLVLTQSPASLAVSPGQRATITCKASQSVDYDGDSYLNWYQQKPGQPPKLLIYDASNLVSGVPARFSGSGSGTDFTLTINPVEANDTANYYCQQSTEDPWTFGQGTKLEIK

SEQ ID NO: 158 - protein, 121 aa, synthetic construct [sequence omitted]

SEQ ID NO: 159 - protein, 106 aa, synthetic construct [sequence omitted]

SEQ ID NO: 160 - protein, 120 aa, synthetic construct
  REGION 1..120: note = Synthetic Construct
QVQLVQSGAEVVKPGASVKVSCKASGYTFTSYYIHWVRQAPGQGLEWIGSIYPGNVNTNYAQKFQGRATLTVDTSISTAYMELSRLRSDDTAVYYCTRSHYGLDWNFDVWGKGTTVTVSS

SEQ ID NO: 161 - protein, 107 aa, synthetic construct
  REGION 1..107: note = Synthetic Construct
DIQMTQSPSSLSASVGDRVTITCQASQNIYVWLNWYQQKPGKAPKLLIYKASNLHTGVPSRFSGSGSGTDFTLTISSLQPEDIATYYCQQGQTYPYTFGQGTKLEIK

SEQ ID NO: 162 - protein, 120 aa, synthetic construct
  REGION 1..120: note = Synthetic Construct
QVQLQESGPGLVKPSQTLSLTCTVSGFSLSDYGVHWVRQPPGKGLEWLGVIWAGGGTNYNPSLKSRKTISKDTSKNQVSLKLSSVTAADTAVYYCARDKGYSYYYSMDYWGQGTTVTVSS

SEQ ID NO: 163 - protein, 111 aa, synthetic construct
  REGION 1..111: note = Synthetic Construct
DIVLTQSPASLAVSPGQRATITCRASESVEYYVTSLMQWYQQKPGQPPKLLIFAASNVESGVPARFSGSGSGTDFTLTINPVEANDVANYYCQQSRKVPYTFGQGTKLEIK

SEQ ID NO: 164 - protein, 120 aa, synthetic construct [sequence omitted]

SEQ ID NO: 165 - protein, 107 aa, synthetic construct [sequence omitted]

SEQ ID NO: 166 - protein, 118 aa, synthetic construct
  REGION 1..118: note = Synthetic Construct
QVQLVQSGAEVKKPGSSVKVSCKASGYIFTNYNIHWVKKSPGQGLEWIGAIYPGNGDAPYSQKFQGKATLTADTSTSTTYMELSSLRSEDTAVYYCVRANWDVAFAYWGQGTLVTVSS

SEQ ID NO: 167 - protein, 106 aa, synthetic construct
  REGION 1..106: note = Synthetic Construct
DIQMTQSPSSLSASVGDRVTITCKASQDIDRYMAWYQDKPGKAPRLLIHDTSTLQSGVPSRFSGSGSGRDYTLTISNLEPEDFATYYCLQYDNLWTFGGGTKVEIK

SEQ ID NO: 168 - protein, 121 aa, synthetic construct [sequence omitted]

SEQ ID NO: 169 - protein, 107 aa, synthetic construct [sequence omitted]

SEQ ID NO: 170 - protein, 123 aa, synthetic construct
  REGION 1..123: note = Synthetic Construct
QVQLQQSGPELVKPGASVKISCKASGYSFTSYWIHWIKQRPGQGLEWIGMIDPSDGETRLNQRFQGRATLTVDESTSTAYMQLRSPTSEDSAVYYCTRLKEYGNYDSFYFDVWGAGTLVTVSS

SEQ ID NO: 171 - protein, 107 aa, synthetic construct
  REGION 1..107: note = Synthetic Construct
DIQMTQSPASLSVSVGDTITLTCHASQNIDVWLSWFQQKPGNIPKLLIYKASNLHTGVPSRFSGSGSGTGFTLTISSLQPEDIATYYCQQAHSYPFTFGGGTKLEIK

SEQ ID NO: 172 - protein, 118 aa, synthetic construct
  REGION 1..118: note = Synthetic Construct
EVQLKESGPGLVAPGGSLSITCTVSGFSLTDSSINWVRQPPGKGLEWLGMIWGDGRIDYADALKSRLSISKDSSKSQVFLEMTSLRTDDTATYYCARDGYFPYAMDFWGQGTSVTVSS

SEQ ID NO: 173 - protein, 111 aa, synthetic construct
  REGION 1..111: note = Synthetic Construct
DIVLTQSPASLAVSLGQRATISCRASESVDSYGQSYMHWYQQKAGQPPKLLIYLASNLESGVPARFSGSGSRTDFTLTIDPVQAEDAATYYCQQNAEDSRTFGGGTKLEIK

SEQ ID NO: 174 - protein, 5 aa, synthetic construct
  REGION 1..5: note = Synthetic Construct
  VARIANT 1..5: note = Can be absent or present, or present in repeats of up to 5 times
GGGGS

SEQ ID NO: 175 - protein, 7 aa, synthetic construct
  REGION 1..7: note = Synthetic Construct
GQPKAAP

SEQ ID NO: 176 - protein, 5 aa, synthetic construct
  REGION 1..5: note = Synthetic Construct
DKTHT

SEQ ID NO: 177 - protein, 6 aa, synthetic construct
  REGION 1..6: note = Synthetic Construct
TKGPSR

SEQ ID NO: 178 - protein, 7 aa, synthetic construct
  REGION 1..7: note = Synthetic Construct
AASTLQS

SEQ ID NO: 179 - protein, 7 aa, synthetic construct
  REGION 1..7: note = Synthetic Construct
KASNLHT